European Patent Application EP 4 375 366 A1, published May 29, 2024. Title: METHOD FOR PRODUCING GLUCOSE AND DERIVATIVES THEREOF BY MEANS OF BIOTRANSFORMATION WITH RECOMBINANT YEAST. Applicant: shen zhen xian jin ji shu yan jiu yuan. Application EP 22845457.5, filed July 22, 2022. The sequence listing filed with the application follows.

SEQUENCE LISTING (44 sequences)

SEQ ID NO: 1 - DNA, 1728 bp, synthetic construct
  source 1..1728: mol_type = other DNA
atgattaagaagttatctttgtgtgctttgtctgttttggccgccttgccagttggtactgttgccttcgctgctgatggcgatatgcaattgcaacaagttttgatgttgtccagacataatttgagagctccattggccgataacggttctgtcttggaacaatctactaagaagtcatggccacaatgggatgttccaggtggtcaattgactactaagggtggtgtcttggaaatctacatgggtaattacaccagacaatggttagctcaacaaggtttagttcaaaatggttcttgtccagattctaacaacgttttcgtttacgctaactcgttacaaagaaccgttgctactgctcaattctttgttaatggtgcttttccaggttgtgatgttgctgtcactcaccaagatgctatgggtactatggacccaattttcaaccctgttattaccgatggctctgaagctttcaacaagcaagctttagctgatatggctgctgctaatggtaaattggctttaaaacctgctttccaaagattggaaaagatcgttgattataaatcttccccagcttgtaataacaaaaaacaatgtgatttgtcatctggtcaaaactctttttctgctgaaaatggtaaagaaccaaatgtttctggtccattgaaggttggtaactctttaattgatgcttttaccttacaatactatgaaggtttcccattggatcaagttgcttggggtcaaattaagactccagaacaatggaaggaattgtctgctataaaaaatggttatcaagatactttgttcacttcaccaactatcgcaagagaagtcgctgccccattagtcgattacatcagatctcaattggtcgaccaagataaggctaatgctccaaaggttactttgatggttggtcatgatagtaacattgcttctttgttatctgctctacaagttaagccatatgaattacctgatacttacgaaaaaactcctattggtggtcaagttgttttcgaaagatggcatgatgctaaaaatgataaggatttgttaaaagtcgaatacgtttaccaaaccgctgatcaattacgtgatgctgatgttttatccttaaagaaccctccaaagagagttaccttgcaattgactggttgtcaaactgatgctaacggttactgttcctgggaccaattctcccaagctttgaattctgctctacaaggtactcctatgcaaccagctgcagctgctaagcctgctgctgctcaacctgattctgatgctgctcctgctgctgctgctgccaactctgctactgataagccagctgataatgctaaagccgataaggctgacgcagataaagctaaggctgagaaagctgaagctgataaggccgctgctgagaaggctaaggcagaaaaagctgacgctgataaagctaaggctgaaaaagctgaagctgataaggctgctgctgaaaaagccaaggctgataaggctgctgctgataaagctgccgctgaaaaagctaaagctgataaagccgctgctgataaagccgctgctgaaaacgctaaagctgaaaaggctgatgctgaaaaggcagctgctgaaaaggctaaggctgataatgctactgcttctcaagctccaactgctgctcaatctaacgatgctaaatctgttgctactgctgctcaataa

SEQ ID NO: 2 - DNA, 600 bp, synthetic construct
  source 1..600: mol_type = other DNA
atgttgtacattttcgatttgggtaacgttattgttgatattgatttcaacagagttttgggtgcttggtctgatttgactagaattccattagcttctttgaagaagtctttccacatgggtgaagctttccatcaacatgaaagaggtgaaatttctgatgaagctttcgctgaagctttgtgtcatgaaatggctttgccattgtcttacgaacaattctctcatggttggcaagctgttttcgttgctttgagacctgaagttattgctattatgcataagttgagagaacaaggtcatagagttgttgttttgtctaacactaatagattgcatactactttctggccagaagaatacccagaaattagagatgctgctgatcatatctacttgtctcaagatttgggtatgagaaagccagaagctagaatctaccaacatgttttgcaagctgaaggtttctctccatctgatactgttttcttcgatgataacgctgataacattgaaggtgctaaccaattgggtattacttctattttagttaaggataagactactattccagattacttcgctaaggttttgtgttaa

SEQ ID NO: 3 - DNA, 998 bp, synthetic construct
  source 1..998: mol_type = other DNA
aaccagggcaaagcaaaataaaagaaacttaatacgttatgccgtaatgaagggctaccaaaaacgataatctcaactgtaaacaggtacaatgcggacccttttgccacaaaacatacatcattcattgccggaaaaagaaagaagtgaagacagcagtgcagccagccatgttgcgccaatctaattatagatgctggtgccctgaggatgtatctggagccagccatggcatcatgcgctaccgccggatgtaaaatccgacacgcaaaagaaaaccttcgaggttgcgcacttcgcccacccatgaaccacacggttagtccaaaaggggcagttcagattccagatgcgggaattagcttgctgccaccctcacctcactaacgctgcggtgtgcggatacttcatgctatttatagacgcgcgtgtcggaatcagcacgcgcaagaaccaaatgggaaaatcggaatgggtccagaactgctttgagtgctggctattggcgtctgatttccgttttgggaatcctttgccgcgcgcccctctcaaaactccgcacaagtcccagaaagcgggaaagaaataaaacgccaccaaaaaaaaaaataaaagccaatcctcgaagcgtgggtggtaggccctggattatcccgtacaagtatttctcaggagtaaaaaaaccgtttgttttggaattccccatttcgcggccacctacgccgctatctttgcaacaactatctgcgataactcagcaaattttgcatattcgtgttgcagtattgcgataatgggagtcttacttccaacataacggcagaaagaaatgtgagaaaattttgcatcctttgcctccgttcaagtatataaagtcggcatgcttgataatctttctttccatcctacattgttctaattattcttattctcctttattctttcctaacataccaagaaattaatcttctgtcattcgcttaaacactatatcaata

SEQ ID NO: 4 - DNA, 401 bp, synthetic construct
  source 1..401: mol_type = other DNA
aaaaagaatcatgattgaatgaagatattatttttttgaattatattttttaaattttatataaagacatggtttttcttttcaactcaaataaagatttataagttacttaaataacatacattttataaggtattctataaaaagagtattatgttattgttaacctttttgtctccaattgtcgtcataacgatgaggtgttgcatttttggaaacgagattgacatagagtcaaaatttgctaaatttgatccctcccatcgcaagataatcttccctcaaggttatcatgattatcaggatggcgaaaggatacgctaaaaattcaataaaaaattcaatataattttcgtttcccaagaactaacttggaaggttatacatgggtacataaatgc

SEQ ID NO: 5 - DNA, 412 bp, synthetic construct
  source 1..412: mol_type = other DNA
atagcttcaaaatgtttctactccttttttactcttccagattttctcggactccgcgcatcgccgtaccacttcaaaacacccaagcacagcatactaaatttcccctctttcttcctctagggtgtcgttaattacccgtactaaaggtttggaaaagaaaaaagagaccgcctcgtttctttttcttcgtcgaaaaaggcaataaaaatttttatcacgtttctttttcttgaaaatttttttttttgatttttttctctttcgatgacctcccattgatatttaagttaataaacggtcttcaatttctcaagtttcagtttcatttttcttgttctattacaactttttttacttcttgctcattagaaagaaagcatagcaatctaatctaagttttaattacaaa

SEQ ID NO: 6 - DNA, 435 bp, synthetic construct
  source 1..435: mol_type = other DNA
taaagtaagagcgctacattggtctacctttttgttcttttacttaaacattagttagttcgttttctttttctcatttttttatgtttcccccccaaagttctgattttataatattttatttcacacaattccatttaacagagggggaatagattctttagcttagaaaattagtgatcaatatatatttgcctttcttttcatcttttcagtgatattaatggtttcgagacactgcaatggccctagttgtctaagaggatagatgttactgtcaaagatgatattttgaatttcaattgacgtaattaatgatactattaataatacagagcgtatatgaagtattgcaaataacatgcacagttcttttgggatgagaatgataatgaaaggcgaaggcgggcgttcagaaaagcgttgcggagtaac

SEQ ID NO: 7 - DNA, 1536 bp, synthetic construct
  source 1..1536: mol_type = other DNA
atggataatccatctactaatgaatcttcaaatatttcttcaattcatctagaatcagctagtaatagaaaaccaactccattaattaagatgattgctgttgcttctattgctgctggtattcaatttggatgggctttacaattgtcattattaactccttatattcaattattaggtgttccacataaatgggctgcaaatatatggttgtgtggtccaatttctggtatgattattcaaccaatagttggttactatagtgatcgtaatagatctaggtttggtagaaggagaccttttattttctttggtgctatagctgttgctgttgctgtatttttgattggttttgctgctgatattggacattcttttggtgacgatttgaagaaaaagactagacctaaagctgttgtaatttttgtttttggtttttggattttagatgttgctaataacatgttgcaaggtccatgtagagcttttattggtgacttagctgctgatgatcatagaagaatgagaacaggtaatgctttattttcatttttcatgactgttggtaatgttttaggttacgctgctggtagttatagaaaattgtttatgatgttaccattcactaaaactgaagcttgtaatgaattttgtgcaaacttaaaaacatgtttctttattgctatatttttgttgattttgttgtctactttcgctttattgtacgttgaagatattccattaccatctattgaatctcaatctcaaactcaaacacaaacacaatctgaacctgaacaacaagtttcttgtttcggtgaaattttaggtgcttttaatggtttacaaaaacctatgtggatgttgatgttagttacagctattaattggattgcttggtttcctttctttttatttgatactgattggatgggtcatgaagtttacggtggaaatccaggagatgatgcttataatagaggtgttagagctggtgcaatgggtttaatgataaacgctgtagttttagctttaatgtctttagcagttgaacctttaggtagatttgtaggcggtgctaaaagattgtggggtattgttaatattattttagcagttggtttagcaatgacaattgttattactaaagctgctcaacatgaaagacatgtatctaatggtaatactccaagtgcaggtatttctgctgctagttttgcatttttcgctttgttaggtattcctttagctattaatttttcagttccttttgctttggcatctatatattcatctgctagtggtgcaggtcaaggtttatccttgggtgttttgaatattgcaattgttgttccacaaatgattgtatctgctttatcaggtccatgggattcattgtttggtggtggtaacttgccagcttttgttgttggtattggtgcagctgttatctctggtgttttagcaattattattttaccaactccaaaagctactgatgttgctaaagttccaattgctggtggttttcattaa

SEQ ID NO: 8 - DNA, 3207 bp, synthetic construct
  source 1..3207: mol_type = other DNA
gagggtctgtccagcgaataagaagaaaacctccttttcggcttttgaagataggttgcagttgtctgcgggcacaaaatgggcaatttttttaatactttttacgtatgagacaagatttttttcgccaattatatcgcatgaagaataaccagagtttttctccgaacgttaagggagttgaagtaaaaataaagaaaggaccaaatgagaatgggtatgcttggtcttagtcttcgaatcaaattctgcttccctgttcatggcaacgtcacctcaattatttggaaagggggggttttccgactttatttgagatgacttgagatgtgtgtcaatgctagtattttggagattaatctcagtacaaaacaatattaaaaagaggtgaattatttttccccccttattttttttttgttagaattgatccaaatgtaaataaacaatcacaaggaaaaaaaaaaaaaaaaaaaaaatagccgccatgaccccggatcgtcggttgtgatagcttcaaaatgtttctactccttttttactcttccagattttctcggactccgcgcatcgccgtaccacttcaaaacacccaagcacagcatactaaatttcccctctttcttcctctagggtgtcgttaattacccgtactaaaggtttggaaaagaaaaaagagaccgcctcgtttctttttcttcgtcgaaaaaggcaataaaaatttttatcacgtttctttttcttgaaaatttttttttttgatttttttctctttcgatgacctcccattgatatttaagttaataaacggtcttcaatttctcaagtttcagtttcatttttcttgttctattacaactttttttacttcttgctcattagaaagaaagcatagcaatctaatctaagttttaattacaaaatggataatccatctactaatgaatcttcaaatatttcttcaattcatctagaatcagctagtaatagaaaaccaactccattaattaagatgattgctgttgcttctattgctgctggtattcaatttggatgggctttacaattgtcattattaactccttatattcaattattaggtgttccacataaatgggctgcaaatatatggttgtgtggtccaatttctggtatgattattcaaccaatagttggttactatagtgatcgtaatagatctaggtttggtagaaggagaccttttattttctttggtgctatagctgttgctgttgctgtatttttgattggttttgctgctgatattggacattcttttggtgacgatttgaagaaaaagactagacctaaagctgttgtaatttttgtttttggtttttggattttagatgttgctaataacatgttgcaaggtccatgtagagcttttattggtgacttagctgctgatgatcatagaagaatgagaacaggtaatgctttattttcatttttcatgactgttggtaatgttttaggttacgctgctggtagttatagaaaattgtttatgatgttaccattcactaaaactgaagcttgtaatgaattttgtgcaaacttaaaaacatgtttctttattgctatatttttgttgattttgttgtctactttcgctttattgtacgttgaagatattccattaccatctattgaatctcaatctcaaactcaaacacaaacacaatctgaacctgaacaacaagtttcttgtttcggtgaaattttaggtgcttttaatggtttacaaaaacctatgtggatgttgatgttagttacagctattaattggattgcttggtttcctttctttttatttgatactgattggatgggtcatgaagtttacggtggaaatccaggagatgatgcttataatagaggtgttagagctggtgcaatgggtttaatgataaacgctgtagttttagctttaatgtctttagcagttgaacctttaggtagatttgtaggcggtgctaaaagattgtggggtattgttaatattattttagcagttggtttagcaatgacaattgttattactaaagctgctcaacatgaaagacatgtatctaatggtaatactccaagtgcaggtatttctgctgctagttttgcatttttcgctttgttaggtattcctttagctattaatttttcagttccttttgctttggcatctatatattcatctgctagtggtgcaggtcaaggtttatccttgggtgttttgaatattgcaattgttgttccacaaatgattgtatctgctttatcaggtccatgggattcattgtttggtggtggtaacttgccagcttttgttgttggtattggtgcagctgttatctctggtgttttagcaattattattttaccaactccaaaagctactgatgttgctaaagttccaattgctggtggttttcattaaattgaattgaattgaaatcgatagatcaatttttttcttttctctttccccatcctttacgctaaaataatagtttattttattttttgaatattttttatttatatacgtatatatagactattatttatcttttaatgattattaagatttttattaaaaaaaaattcgctcctcttttaatgcctttatgcagtttttttttcccattcgatatttctatgttcgggttcagcgtattttaagtttaataactcgaaaattctgcgttcgttagctaatttttccggcagaaagattttcgctacccgaaagtttttccggcaagctaaatggaaaaaggaaagattattgaaagagaaagaaagaaaaaaaaaaaatgtacacccagacatcgggcttccacaatttcggctctattgttttccatctctcgcaacggcgggattcctctatggcgtgtgatgtctgtatctgttacttaatccagaaactggcacttgacccaactctgccacgtgggtcgttttgccatcgacagattgggagattttcatagtagaattcagcatgatagctacgtaaatgtgttccgcaccgtcacaaagtgttttctactgttctttcttctttcgttcattcagttgagttgagtgagtgctttgttcaatggatcttagctaaaatgcatattttttctcttggtaaatgaatgcttgtgatgtcttccaagtgatttcctttccttc

SEQ ID NO: 9 - DNA, 735 bp, synthetic construct
  source 1..735: mol_type = other DNA
atgagacaattgttgttgatttctgatttggataacacttgggtcggcgatcaacaagctttggaacatttgcaagaatacttgggtgacagaagaggtaacttttacttggcttacgctactggtagatcctaccactctgctagagaattgcaaaagcaagttggtttgatggaaccagattactggttgactgctgttggttctgaaatctatcatccagaaggtttagatcaacactgggctgattacttgtccgaacattggcaaagagatattttgcaagctattgctgatggttttgaagccttgaagccacaatctccattagaacaaaacccatggaaaatttcttatcacttagatccacaagcttgtccaaccgttattgatcaattgaccgaaatgttgaaggaaactggtattccagttcaagttattttctcctctggtaaagatgttgacttgttaccacaacgttctaataagggtaacgctactcaatacttgcaacaacatttggctatggaaccatctcaaactttggtttgtggtgactctggtaacgatattggtttgtttgaaacttctgctagaggtgttattgttagaaacgctcaaccagaattgttgcattggtacgatcaatggggtgactctagacattacagagctcaatcttctcatgctggtgctatcttggaagctattgctcattttgatttcttgtcttaa

SEQ ID NO: 10 - DNA, 2163 bp, synthetic construct
  source 1..2163: mol_type = other DNA
atgtcttactcctctaagtacattttgttgatttctgttcatggtttgattagaggtgaaaacttagaattaggtagagatgctgatactggtggtcaaaccaaatacgttttggaattagctagagctctagttaaaaatccacaagtagctagagttgatcttttgacaagattaattaaggatccaaaagttgatgctgattatgcacaacctagagaattaattggtgacagagctcaaattgttagaattgaatgtggtcctgaagaatatatcgctaaagaaatgttgtgggattacttagataacttcgctgatcacgctttagattacctaaaggaacaacctgaattgcctgatgttattcattctcactacgctgatgctggttacgttggtactagattgtcacaccaattgggtatcccattagttcatactggtcactctttaggtcgttctaagagaactagactattattgtctggtattaaggctgatgaaattgaatctagatacaatatggccagacgtattaacgctgaagaagaaactttaggttcagctgccagagtcattacctctactcaccaagaaatcgcagaacaatatgctcaatacgattattaccaaccagatcaaatgcttgtcattccaccaggtactgatttggaaaagttttacccaccaaaaggtaatgaatgggaaaccccaattgttcaagaattacaaagattcttgagacacccaagaaagccaattatcttggccttgtctcgtccagatccaagaaagaacattcataagttgattgcagcttatggccaatctccacaactacaagcccaagctaacctagtcatcgttgctggtaaccgggacgacattactgatttggatcaaggtccacgtgaagtgttgaccgatttgttgttaacaattgataggtacgatttgtatggcaaggttgcttatcctaagcaaaaccaagctgaggacgtttatgctttattccgtcttactgctttgtcccaaggtgtattcattaatccagctttgactgaaccttttggtttgactttgattgaagccgctgcttgtggtgtccccattgttgctactgaagatggcggtcctgttgatatcatcaagaattgtcaaaatggttatttgattaacccgttggatgaagttgatatcgcagataagttattgaaagttttgaacgataagcaacaatggcaattcttatcagaatctggtttggaaggcgttaaaaggcactattcttggccatcccatgttgaatcttatcttgaagctattaacgcgttgactcaacaaacttcagttttgaaacgttctgacttaaaaagaagaagaaccttgtactacaacggtgccttggttaccagtttagatcaaaacttgttgggtgctttacaaggtggtttacctggcgacagacaaactttggatgaattgttagaagttttgtaccaacatagaaagaacgtcggtttttgtattgccacaggtagaaggttggattctgtcttgaagattttgagagaatacagaatcccacaacctgatatgttgatcacctctatgggtactgagatctactcctctcctgatttgattcctgatcaatcttggcgtaatcatattgactatttgtggaacagaaatgcaattgttagaattttaggtgaattgccaggcttagctttgcaaccaaaggaagaactatctgcttacaagatcagttacttttacgacgccgctattgcaccaaacctagaagaaattagacaattgttacataaaggtgaacaaaccgtgaacactatcattagctttggtcaattcttggatattttgccaattagagcttctaagggttacgctgtcagatggttatcgcaacaatggaatattccattagaacatgtttttactgctggtggttcaggcgctgatgaagatatgatgagaggtaacactttgtctgttgtagttgctaatagacatcacgaagaattgtctaatctaggtgaaattgaaccaatctacttctccgaaaagagatacgctgctggtattttggatggtttggctcactacagattcttcgaattgttagacccagtttaa

SEQ ID NO: 11 - DNA, 5255 bp, synthetic construct
  source 1..5255: mol_type = other DNA
caacttgctctcgaagtggtcgcgaatttcttatgatttatgatttttattattaaataagttataaaaaaaataagtgtatacaaattttaaagtgactcttaggttttaaaacgaaaattcttattcttgagtaactctttcctgtaggtcaggttgctttctcaggtatagcatgaggtcgctcttattgaccacacctctaccggcatgccgagcaaatgcctgcaaatcgctccccatttcacccaattgtagatatgcttaaactgggtctaacaattcgaagaatctgtagtgagccaaaccatccaaaataccagcagcgtatctcttttcggagaagtagattggttcaatttcacctagattagacaattcttcgtgatgtctattagcaactacaacagacaaagtgttacctctcatcatatcttcatcagcgcctgaaccaccagcagtaaaaacatgttctaatggaatattccattgttgcgataaccatctgacagcgtaacccttagaagctctaattggcaaaatatccaagaattgaccaaagctaatgatagtgttcacggtttgttcacctttatgtaacaattgtctaatttcttctaggtttggtgcaatagcggcgtcgtaaaagtaactgatcttgtaagcagatagttcttcctttggttgcaaagctaagcctggcaattcacctaaaattctaacaattgcatttctgttccacaaatagtcaatatgattacgccaagattgatcaggaatcaaatcaggagaggagtagatctcagtacccatagaggtgatcaacatatcaggttgtgggattctgtattctctcaaaatcttcaagacagaatccaaccttctacctgtggcaatacaaaaaccgacgttctttctatgttggtacaaaacttctaacaattcatccaaagtttgtctgtcgccaggtaaaccaccttgtaaagcacccaacaagttttgatctaaactggtaaccaaggcaccgttgtagtacaaggttcttcttctttttaagtcagaacgtttcaaaactgaagtttgttgagtcaacgcgttaatagcttcaagataagattcaacatgggatggccaagaatagtgccttttaacgccttccaaaccagattctgataagaattgccattgttgcttatcgttcaaaactttcaataacttatctgcgatatcaacttcatccaacgggttaatcaaataaccattttgacaattcttgatgatatcaacaggaccgccatcttcagtagcaacaatggggacaccacaagcagcggcttcaatcaaagtcaaaccaaaaggttcagtcaaagctggattaatgaatacaccttgggacaaagcagtaagacggaataaagcataaacgtcctcagcttggttttgcttaggataagcaaccttgccatacaaatcgtacctatcaattgttaacaacaaatcggtcaacacttcacgtggaccttgatccaaatcagtaatgtcgtcccggttaccagcaacgatgactaggttagcttgggcttgtagttgtggagattggccataagctgcaatcaacttatgaatgttctttcttggatctggacgagacaaggccaagataattggctttcttgggtgtctcaagaatctttgtaattcttgaacaattggggtttcccattcattaccttttggtgggtaaaacttttccaaatcagtacctggtggaatgacaagcatttgatctggttggtaataatcgtattgagcatattgttctgcgatttcttggtgagtagaggtaatgactctggcagctgaacctaaagtttcttcttcagcgttaatacgtctggccatattgtatctagattcaatttcatcagccttaataccagacaataatagtctagttctcttagaacgacctaaagagtgaccagtatgaactaatgggatacccaattggtgtgacaatctagtaccaacgtaaccagcatcagcgtagtgagaatgaataacatcaggcaattcaggttgttcctttaggtaatctaaagcgtgatcagcgaagttatctaagtaatcccacaacatttctttagcgatatattcttcaggaccacattcaattctaacaatttgagctctgtcaccaattaattctctaggttgtgcataatcagcatcaacttttggatccttaattaatcttgtcaaaagatcaactctagctacttgtggatttttaactagagctctagctaattccaaaacgtatttggtttgaccaccagtatcagcatctctacctaattctaagttttcacctctaatcaaaccatgaacagaaatcaacaaaatgtacttagaggagtaagacattttgtttgtttatgtgtgtttattcgaaactaagttcttggtgttttaaaactaaaaaaaagactaactataaaagtagaatttaagaagtttaagaaatagatttacagaattacaatcaatacctaccgtctttatatacttattagtcaagtaggggaataatttcagggaactggtttaaaccttttttttcagctttttccaaatcagagagagcagaaggtaatagaaggtgtaagaaaatgagatagatacatgcgtgggtcaattgccttgtgtcatcatttactccaggcaggttgcatcactccattgaggttgtgcccgttttttgcctgtttgtgccctgttctctgtagttgcgctaagagaatggacctatgaactgatggttggtgaagaaaacaatattttggtgctgggattctttttttttctggatgccagcttaaaaagcgggctccattatatttagtggatgccaggaataaacctgttcacccaagcaccatcagtgttatatattctgtgtaacccgccccctattttggcatgtacgggttacagcagaattaaaaggctaattttttgactaaataaagttaggaaaatcactactattaattatttacgtattctttgaaatggcagtattgataatgataaactcgaaaccagggcaaagcaaaataaaagaaacttaatacgttatgccgtaatgaagggctaccaaaaacgataatctcaactgtaaacaggtacaatgcggacccttttgccacaaaacatacatcattcattgccggaaaaagaaagaagtgaagacagcagtgcagccagccatgttgcgccaatctaattatagatgctggtgccctgaggatgtatctggagccagccatggcatcatgcgctaccgccggatgtaaaatccgacacgcaaaagaaaaccttcgaggttgcgcacttcgcccacccatgaaccacacggttagtccaaaaggggcagttcagattccagatgcgggaattagcttgctgccaccctcacctcactaacgctgcggtgtgcggatacttcatgctatttatagacgcgcgtgtcggaatcagcacgcgcaagaaccaaatgggaaaatcggaatgggtccagaactgctttgagtgctggctattggcgtctgatttccgttttgggaatcctttgccgcgcgcccctctcaaaactccgcacaagtcccagaaagcgggaaagaaataaaacgccaccaaaaaaaaaaataaaagccaatcctcgaagcgtgggtggtaggccctggattatcccgtacaagtatttctcaggagtaaaaaaaccgtttgttttggaattccccatttcgcggccacctacgccgctatctttgcaacaactatctgcgataactcagcaaattttgcatattcgtgttgcagtattgcgataatgggagtcttacttccaacataacggcagaaagaaatgtgagaaaattttgcatcctttgcctccgttcaagtatataaagtcggcatgcttgataatctttctttccatcctacattgttctaattattcttattctcctttattctttcctaacataccaagaaattaatcttctgtcattcgcttaaacactatatcaataatgagacaattgttgttgatttctgatttggataacacttgggtcggcgatcaacaagctttggaacatttgcaagaatacttgggtgacagaagaggtaacttttacttggcttacgctactggtagatcctaccactctgctagagaattgcaaaagcaagttggtttgatggaaccagattactggttgactgctgttggttctgaaatctatcatccagaaggtttagatcaacactgggctgattacttgtccgaacattggcaaagagatattttgcaagctattgctgatggttttgaagccttgaagccacaatctccattagaacaaaacccatggaaaatttcttatcacttagatccacaagcttgtccaaccgttattgatcaattgaccgaaatgttgaaggaaactggtattccagttcaagttattttctcctctggtaaagatgttgacttgttaccacaacgttctaataagggtaacgctactcaatacttgcaacaacatttggctatggaaccatctcaaactttggtttgtggtgactctggtaacgatattggtttgtttgaaacttctgctagaggtgttattgttagaaacgctcaaccagaattgttgcattggtacgatcaatggggtgactctagacattacagagctcaatcttctcatgctggtgctatcttggaagctattgctcattttgatttcttgtcttaagttaattcaaattaattgatatagttttttaatgagtattgaatctgtttagaaataatggaatattatttttatttatttatttatattattggtcggctcttttcttctgaaggtcaatgacaaaatgatatgaaggaaataatgatttctaaaattttacaacgtaagatatttttacaaaagcctagctcatcttttgtcatgcactattttactcacgcttgaaattaacggccagtccactgcggagtcatttcaaagtcatcctaatcgatctatcgtttttgatagctcattttggagttcgcgattgtcttctgttattcacaactgttttaatttttatttcattctggaactcttcgagttctttgtaaagtctttcatagtagcttactcctgcataatcggcctcac

SEQ ID NO: 12 - DNA, 1500 bp, synthetic construct
  source 1..1500: mol_type = other DNA
atgtccactaagaagcacaccaaaacacattccacttatgcattcgagagcaacacaaacagcgttgctgcctcacaaatgagaaacgccttaaacaagttggcggactctagtaaacttgacgatgctgctcgcgctaagtttgagaacgaactggattcgtttttcacgcttttcaggagatatttggtagagaagtcttctagaaccaccttggaatgggacaagatcaagtctcccaacccggatgaagtggttaagtatgaaattatttctcagcagcccgagaatgtctcaaacctttccaaattggctgttttgaagttgaacggtgggctgggtacctccatgggctgcgttggccctaaatctgttattgaagtgagagagggaaacacctttttggatttgtctgttcgtcaaattgaatacttgaacagacagtacgatagcgacgtgccattgttattgatgaattctttcaacactgacaaggatacggaacacttgattaagaagtattccgctaacagaatcagaatcagatctttcaatcaatccaggttcccaagagtctacaaggattctttattgcctgtccccaccgaatacgattctccactggatgcttggtatccaccaggtcacggtgatttgtttgaatctttacacgtatctggtgaactggatgccttaattgcccaaggaagagaaatattatttgtttctaacggtgacaacttgggtgctaccgtcgacttaaaaattttaaaccacatgatcgagactggtgccgaatatataatggaattgactgataagaccagagccgatgttaaaggtggtactttgatttcttacgatggtcaagtccgtttattggaagtcgcccaagttccaaaagaacacattgacgaattcaaaaatatcagaaagtttaccaacttcaacacgaataacttatggatcaatctgaaagcagtaaagaggttgatcgaatcgagcaatttggagatggaaatcattccaaaccaaaaaactataacaagagacggtcatgaaattaatgtcttacaattagaaaccgcttgtggtgctgctatcaggcattttgatggtgctcacggtgttgtcgttccaagatcaagattcttgcctgtcaagacctgttccgatttgttgctggttaaatcagatctattccgtctggaacacggttctttgaagttagacccatcccgttttggtccaaacccattaatcaagttgggctcgcatttcaaaaaggtttctggttttaacgcaagaatccctcacatcccaaaaatcgtcgagctagatcatttgaccatcactggtaacgtctttttaggtaaagatgtcactttgaggggtactgtcatcatcgtttgctccgacggtcataaaatcgatattccaaacggctccatattggaaaatgttgtcgttactggtaatttgcaaatcttggaacattga

SEQ ID NO: 13 - DNA, 1296 bp, synthetic construct
  source 1..1296: mol_type = other DNA
atggttagtttagagaagaacgatcacttaatgttggcgcgccagctgccattgaaatctgttgccctgatactggcgggaggacgtggtacccgcctgaaggatttaaccaataagcgagcaaaaccggccgtacacttcggcggtaagttccgcattatcgactttgcgctgtctaactgcatcaactccgggatcaaacgtatgggcgtgatcacccagtaccagtcccacactctggtgcagcacattcagcgcggctggtcattcttcaatgaagaaatgaacgagtttgtcgatctgctgccagcacagcagagaatgaaaggggaaaactggtatcgcggcaccgcagatgcggtcacccaaaacctcgacattatccgtcgttataaagcggaatacgtggtgatcctggcgggcgaccatatctacaagcaagactactcgcgtatgcttatcgatcacgtcgaaaaaggtgtacgttgtaccgttgtttgtatgccagtaccgattgaagaagcctccgcatttggcgttatggcggttgatgagaacgataaaactatcgaattcgtggaaaaacctgctaacccgccgtcaatgccgaacgatccgagcaaatctctggcgagtatgggtatctacgtctttgacgccgactatctgtatgaactgctggaagaagacgatcgcgatgagaactccagccacgactttggcaaagatttgattcccaagatcaccgaagccggtctggcctatgcgcacccgttcccgctctcttgcgtacaatccgacccggatgccgagccgtactggcgcgatgtgggtacgctggaagcttactggaaagcgaacctcgatctggcctctgtggtggataaactggatatgtacgatcgcaattggccaattcgcacctacaatgaatcattaccgccagcgaaattcgtgcaggatcgctccggtagccacgggatgacccttaactcactggtttccgatggttgtgtgatctccggttcggtggtggtgcagtccgttctgttctcgcgcgttcgcgtgaattcattctgcaacattgattccgccgtattgttaccggaagtatgggtaggtcgctcgtgccgtctgcgccgctgcgtcatcgatcgtgcttgtgttattccggaaggcatggtgattggtgaaaacgcagaggaagatgcacgtcgtttctatcgttcagaagaaggcatcgtgctggtaacgcgcgaaatgctacggaagttagggcataaacaggagcgataa

SEQ ID NO: 14 - DNA, 4670 bp, synthetic construct
  source 1..4670: mol_type = other DNA
gcgagagccgacatacgagacgcatttatgtacccatgtataaccttccaagttagttcttgggaaacgaaaattatattgaattttttattgaatttttagcgtatcctttcgccatcctgataatcatgataaccttgagggaagattatcttgcgatgggagggatcaaatttagcaaattttgactctatgtcaatctcgtttccaaaaatgcaacacctcatcgttatgacgacaattggagacaaaaaggttaacaataacataatactctttttatagaataccttataaaatgtatgttatttaagtaacttataaatctttatttgagttgaaaagaaaaaccatgtctttatataaaatttaaaaaatataattcaaaaaaataatatcttcattcaatcatgattctttttttatcgctcctgtttatgccctaacttccgtagcatttcgcgcgttaccagcacgatgccttcttctgaacgatagaaacgacgtgcatcttcctctgcgttttcaccaatcaccatgccttccggaataacacaagcacgatcgatgacgcagcggcgcagacggcacgagcgacctacccatacttccggtaacaatacggcggaatcaatgttgcagaatgaattcacgcgaacgcgcgagaacagaacggactgcaccaccaccgaaccggagatcacacaaccatcggaaaccagtgagttaagggtcatcccgtggctaccggagcgatcctgcacgaatttcgctggcggtaatgattcattgtaggtgcgaattggccaattgcgatcgtacatatccagtttatccaccacagaggccagatcgaggttcgctttccagtaagcttccagcgtacccacatcgcgccagtacggctcggcatccgggtcggattgtacgcaagagagcgggaacgggtgcgcataggccagaccggcttcggtgatcttgggaatcaaatctttgccaaagtcgtggctggagttctcatcgcgatcgtcttcttccagcagttcatacagatagtcggcgtcaaagacgtagatacccatactcgccagagatttgctcggatcgttcggcattgacggcgggttagcaggtttttccacgaattcgatagttttatcgttctcatcaaccgccataacgccaaatgcggaggcttcttcaatcggtactggcatacaaacaacggtacaacgtacacctttttcgacgtgatcgataagcatacgcgagtagtcttgcttgtagatatggtcgcccgccaggatcaccacgtattccgctttataacgacggataatgtcgaggttttgggtgaccgcatctgcggtgccgcgataccagttttcccctttcattctctgctgtgctggcagcagatcgacaaactcgttcatttcttcattgaagaatgaccagccgcgctgaatgtgctgcaccagagtgtgggactggtactgggtgatcacgcccatacgtttgatcccggagttgatgcagttagacagcgcaaagtcgataatgcggaacttaccgccgaagtgtacggccggttttgctcgcttattggttaaatccttcaggcgggtaccacgtcctcccgccagtatcagggcaacagatttcaatggcagctggcgcgccaacattaagtgatcgttcttctctaaactaaccattttgtaattaaaacttagattagattgctatgctttctttctaatgagcaagaagtaaaaaaagttgtaatagaacaagaaaaatgaaactgaaacttgagaaattgaagaccgtttattaacttaaatatcaatgggaggtcatcgaaagagaaaaaaatcaaaaaaaaaaattttcaagaaaaagaaacgtgataaaaatttttattgcctttttcgacgaagaaaaagaaacgaggcggtctcttttttcttttccaaacctttagtacgggtaattaacgacaccctagaggaagaaagaggggaaatttagtatgctgtgcttgggtgttttgaagtggtacggcgatgcgcggagtccgagaaaatctggaagagtaaaaaaggagtagaaacattttgaagctatacgcggcgttatgtcactaacgacgtgcaccaacttgcggaaagtggaatcccgttccaaaactggcatccactaattgatacatctacacaccgcacgccttttttctgaagcccactttcgtggactttgccatatgcaaaattcatgaagtgtgataccaagtcagcatacacctcactagggtagtttctttggttgtattgatcatttggttcatcgtggttcattaattttttttctccattgctttctggctttgatcttactatcatttggatttttgtcgaaggttgtagaattgtatgtgacaagtggcaccaagcatatataaaaaaaaaaagcattatcttcctaccagagttgattgttaaaaacgtatttatagcaaacgcaattgtaattaattcttattttgtatcttttcttcccttgtctcaatcttttatttttattttatttttcttttcttagtttctttcataacaccaagcaactaatactataacatacaataataatgtccactaagaagcacaccaaaacacattccacttatgcattcgagagcaacacaaacagcgttgctgcctcacaaatgagaaacgccttaaacaagttggcggactctagtaaacttgacgatgctgctcgcgctaagtttgagaacgaactggattcgtttttcacgcttttcaggagatatttggtagagaagtcttctagaaccaccttggaatgggacaagatcaagtctcccaacccggatgaagtggttaagtatgaaattatttctcagcagcccgagaatgtctcaaacctttccaaattggctgttttgaagttgaacggtgggctgggtacctccatgggctgcgttggccctaaatctgttattgaagtgagagagggaaacacctttttggatttgtctgttcgtcaaattgaatacttgaacagacagtacgatagcgacgtgccattgttattgatgaattctttcaacactgacaaggatacggaacacttgattaagaagtattccgctaacagaatcagaatcagatctttcaatcaatccaggttcccaagagtctacaaggattctttattgcctgtccccaccgaatacgattctccactggatgcttggtatccaccaggtcacggtgatttgtttgaatctttacacgtatctggtgaactggatgccttaattgcccaaggaagagaaatattatttgtttctaacggtgacaacttgggtgctaccgtcgacttaaaaattttaaaccacatgatcgagactggtgccgaatatataatggaattgactgataagaccagagccgatgttaaaggtggtactttgatttcttacgatggtcaagtccgtttattggaagtcgcccaagttccaaaagaacacattgacgaattcaaaaatatcagaaagtttaccaacttcaacacgaataacttatggatcaatctgaaagcagtaaagaggttgatcgaatcgagcaatttggagatggaaatcattccaaaccaaaaaactataacaagagacggtcatgaaattaatgtcttacaattagaaaccgcttgtggtgctgctatcaggcattttgatggtgctcacggtgttgtcgttccaagatcaagattcttgcctgtcaagacctgttccgatttgttgctggttaaatcagatctattccgtctggaacacggttctttgaagttagacccatcccgttttggtccaaacccattaatcaagttgggctcgcatttcaaaaaggtttctggttttaacgcaagaatccctcacatcccaaaaatcgtcgagctagatcatttgaccatcactggtaacgtctttttaggtaaagatgtcactttgaggggtactgtcatcatcgtttgctccgacggtcataaaatcgatattccaaacggctccatattggaaaatgttgtcgttactggtaatttgcaaatcttggaacattgaaggtgcggcttgcaatcccttttttactttcaattctccgttaggttatttattctactacacgcagtttttttttttcaatgggttatatatctctaatatatacacatttatatgtttagacttatacagaagcaaaaaaaaatgcaaaagaagcttagtgttcataattcttcactcacgtcatgttatatatttgttaagcgtagcttcagtatatatagagattttcctttggcggggtaagggtctgtgaactttagggaaatagaataaacgtaagttaaaggtgacaagctcggatcgtcatctttcaattatcaccccaaaagatattgtaaaaaagcaagttcaatctcgtttgttacatttgtcccgtatttctactaattcaggcaaaaaaggaaagtcctacagcaaaagaggcaaaagtacagtatggaaatcgatggcaacactctggtgttcataatagtgatccttttcctatttttctcctctgtgtccgcgtttctaaggc

SEQ ID NO: 15 - DNA, 4685 bp, synthetic construct
  source 1..4685: mol_type = other DNA
gcgagagccgacatacgagacgcatttatgtacccatgtataaccttccaagttagttcttgggaaacgaaaattatattgaattttttattgaatttttagcgtatcctttcgccatcctgataatcatgataaccttgagggaagattatcttgcgatgggagggatcaaatttagcaaattttgactctatgtcaatctcgtttccaaaaatgcaacacctcatcgttatgacgacaattggagacaaaaaggttaacaataacataatactctttttatagaataccttataaaatgtatgttatttaagtaacttataaatctttatttgagttgaaaagaaaaaccatgtctttatataaaatttaaaaaatataattcaaaaaaataatatcttcattcaatcatgattctttttttatcgctcctgtttatgccctaacttccgtagcatttcgcgcgttaccagcacgatgccttcttctgaacgatagaaacgacgtgcatcttcctctgcgttttcaccaatcaccatgccttccggaataacacaagcacgatcgatgacgcagcggcgcagacggcacgagcgacctacccatacttccggtaacaatacggcggaatcaatgttgcagaatgaattcacgcgaacgcgcgagaacagaacggactgcaccaccaccgaaccggagatcacacaaccatcggaaaccagtgagttaagggtcatcccgtggctaccggagcgatcctgcacgaatttcgctggcggtaatgattcattgtaggtgcgaattggccaattgcgatcgtacatatccagtttatccaccacagaggccagatcgaggttcgctttccagtaagcttccagcgtacccacatcgcgccagtacggctcggcatccgggtcggattgtacgcaagagagcgggaacgggtgcgcataggccagaccggcttcggtgatcttgggaatcaaatctttgccaaagtcgtggctggagttctcatcgcgatcgtcttcttccagcagttcatacagatagtcggcgtcaaagacgtagatacccatactcgccagagatttgctcggatcgttcggcattgacggcgggttagcaggtttttccacgaattcgatagttttatcgttctcatcaaccgccataacgccaaatgcggaggcttcttcaatcggtactggcatacaaacaacggtacaacgtacacctttttcgacgtgatcgataagcatacgcgagtagtcttgcttgtagatatggtcgcccgccaggatcaccacgtattccgctttataacgacggataatgtcgaggttttgggtgaccgcatctgcggtgccgcgataccagttttcccctttcattctctgctgtgctggcagcagatcgacaaactcgttcatttcttcattgaagaatgaccagccgcgctgaatgtgctgcaccagagtgtgggactggtactgggtgatcacgcccatacgtttgatcccggagttgatgcagttagacagcgcaaagtcgataatgcggaacttaccgccgaagtgtacggccggttttgctcgcttattggttaaatccttcaggcgggtaccacgtcctcccgccagtatcagggcaacagatttcaatggcagctggcgcgccaacattaagtgatcgttcttctctaaactaaccattttgtaattaaaacttagattagattgctatgctttctttctaatgagcaagaagtaaaaaaagttgtaatagaacaagaaaaatgaaactgaaacttgagaaattgaagaccgtttattaacttaaatatcaatgggaggtcatcgaaagagaaaaaaatcaaaaaaaaaaattttcaagaaaaagaaacgtgataaaaatttttattgcctttttcgacgaagaaaaagaaacgaggcggtctcttttttcttttccaaacctttagtacgggtaattaacgacaccctagaggaagaaagaggggaaatttagtatgctgtgcttgggtgttttgaagtggtacggcgatgcgcggagtccgagaaaatctggaagagtaaaaaaggagtagaaacattttgaagctatacgcggcgttatgtcactaacgacgtgcaccaacttgcggaaagtggaatcccgttccaaaactggcatccactaattgatacatctacacaccgcacgccttttttctgaagcccactttcgtggactttgccatatgcaaaattcatgaagtgtgataccaagtcagcatacacctcactagggtagtttctttggttgtattgatcatttggttcatcgtggttcattaattttttttctccattgctttctggctttgatcttactatcatttggatttttgtcgaaggttgtagaattgtatgtgacaagtggcaccaagcatatataaaaaaaaaaagcattatcttcctaccagagttgattgttaaaaacgtatttatagcaaacgcaattgtaattaattcttattttgtatcttttcttcccttgtctcaatcttttatttttattttatttttcttttcttagtttctttcataacaccaagcaactaatactataacatacaataataatgtccactaagaagcacaccaaaacacattccacttatgcattcgagagcaacacaaacagcgttgctgcctcacaaatgagaaacgccttaaacaagttggcggactctagtaaacttgacgatgctgctcgcgctaagtttgagaacgaactggattcgtttttcacgcttttcaggagatatttggtagagaagtcttctagaaccaccttggaatgggacaagatcaagtctcccaacccggatgaagtggttaagtatgaaattatttctcagcagcccgagaatgtctcaaacctttccaaattggctgttttgaagttgaacggtgggctgggtacctccatgggctgcgttggccctaaatctgttattgaagtgagagagggaaacacctttttggatttgtctgttcgtcaaattgaatacttgaacagacagtacgatagcgacgtgccattgttattgatgaattctttcaacactgacaaggatacggaacacttgattaagaagtattccgctaacagaatcagaatcagatctttcaatcaatccaggttcccaagagtctacaaggattctttattgcctgtccccaccgaatacgattctccactggatgcttggtatccaccaggtcacggtgatttgtttgaatctttacacgtatctggtgaactggatgccttaattgcccaaggaagagaaatattatttgtttctaacggtgacaacttgggtgctaccgtcgacttaaaaattttaaaccacatgatcgagactggtgccgaatatataatggaattgactgataagaccagagccgatgttaaaggtggtactttgatttcttacgatggtcaagtccgtttattggaagtcgcccaagttccaaaagaacacattgacgaattcaaaaatatcagaaagtttaccaacttcaacacgaataacttatggatcaatctgaaagcagtaaagaggttgatcgaatcgagcaatttggagatggaaatcattccaaaccaaaaaactataacaagagacggtcatgaaattaatgtcttacaattagaaaccgcttgtggtgctgctatcaggcattttgatggtgctcacggtgttgtcgttccaagatcaagattcttgcctgtcaagacctgttccgatttgttgctggttaaatcagatctattccgtctggaacacggttctttgaagttagacccatcccgttttggtccaaacccattaatcaagttgggctcgcatttcaaaaaggtttctggttttaacgcaagaatccctcacatcccaaaaatcgtcgagctagatcatttgaccatcactggtaacgtctttttaggtaaagatgtcactttgaggggtactgtcatcatcgtttgctccgacggtcataaaatcgatattccaaacggctccatattggaaaatgttgtcgttactggtaatttgcaaatcttggaacattgaaggtgcggcttgcaatcccttttttactttcaattctccgttaggttatttattctactacacgcagtttttttttttcaatgggttatatatctctaatatatacacatttatatgtttagacttatacagaagcaaaaaaaaatgcaaaagaagcttagtgttcataattcttcactcacgtcatgttatatatttgttaagcgtagcttcagtatatatagagattttcctttggcggggtaagggtctgtgaactttagggaaatagaataaacgtaagttaaaggtgacaagctcggatcgtcatctttcaattatcaccccaaaagatattgtaaaaaagcaagttcaatctcgtttgttacatttgtcccgtatttctactaattcaggcaaaaaaggaaagtcctacagcaaaagaggcaaaagtacagtatggaaatcgatggcaacactctggtgttcataatagtgatccttttcctatttttctcctcgcgaatttcttatgatttatgatttttattattaa

SEQ ID NO: 16 - DNA, 7273 bp, synthetic construct
  source 1..7273: mol_type = other DNA
ataacaccaagcaactaatactataacatacaataataatgtccactaagaagcacaccaaaacacattccacttatgcattcgagagcaacacaaacagcgttgctgcctcacaaatgagaaacgccttaaacaagttggcggactctagtaaacttgacgatgctgctcgcgctaagtttgagaacgaactggattcgtttttcacgcttttcaggagatatttggtagagaagtcttctagaaccaccttggaatgggacaagatcaagtctcccaacccggatgaagtggttaagtatgaaattatttctcagcagcccgagaatgtctcaaacctttccaaattggctgttttgaagttgaacggtgggctgggtacctccatgggctgcgttggccctaaatctgttattgaagtgagagagggaaacacctttttggatttgtctgttcgtcaaattgaatacttgaacagacagtacgatagcgacgtgccattgttattgatgaattctttcaacactgacaaggatacggaacacttgattaagaagtattccgctaacagaatcagaatcagatctttcaatcaatccaggttcccaagagtctacaaggattctttattgcctgtccccaccgaatacgattctccactggatgcttggtatccaccaggtcacggtgatttgtttgaatctttacacgtatctggtgaactggatgccttaattgcccaaggaagagaaatattatttgtttctaacggtgacaacttgggtgctaccgtcgacttaaaaattttaaaccacatgatcgagactggtgccgaatatataatggaattgactgataagaccagagccgatgttaaaggtggtactttgatttcttacgatggtcaagtccgtttattggaagtcgcccaagttccaaaagaacacattgacgaattcaaaaatatcagaaagtttaccaacttcaacacgaataacttatggatcaatctgaaagcagtaaagaggttgatcgaatcgagcaatttggagatggaaatcattccaaaccaaaaaactataacaagagacggtcatgaaattaatgtcttacaattagaaaccgcttgtggtgctgctatcaggcattttgatggtgctcacggtgttgtcgttccaagatcaagattcttgcctgtcaagacctgttccgatttgttgctggttaaatcagatctattccgtctggaacacggttctttgaagttagacccatcccgttttggtccaaacccattaatcaagttgggctcgcatttcaaaaaggtttctggttttaacgcaagaatccctcacatcccaaaaatcgtcgagctagatcatttgaccatcactggtaacgtctttttaggtaaagatgtcactttgaggggtactgtcatcatcgtttgctccgacggtcataaaatcgatattccaaacggctccatattggaaaatgttgtcgttactggtaatttgcaaatcttggaacattgaaggtgcggcttgcaatcccttttttactttcaattctccgttaggttatttattctactacacgcagtttttttttttcaatgggttatatatctctaatatatacacatttatatgtttagacttatacagaagcaaaaaaaaatgcaaaagaagcttagtgttcataattcttcactcacgtcatgttatatatttgttaagcgtagcttcagtatatatagagattttcctttggcggggtaagggtctgtgaactttagggaaatagaataaacgtaagttaaaggtgacaagctcggatcgtcatctttcaattatcaccccaaaagatattgtaaaaaagcaagttcaatctcgtttgttacatttgtcccgtatttctactaattcaggcaaaaaaggaaagtcctacagcaaaagaggcaaaagtacagtatggaaatcgatggcaacactctggtgttcataatagtgatccttttcctatttttctcctcgcgaatttcttatgatttatgatttttattattaaataagttataaaaaaaataagtgtatacaaattttaaagtgactcttaggttttaaaacgaaaattcttattcttgagtaactctttcctgtaggtcaggttgctttctcaggtatagcatgaggtcgctcttattgaccacacctctaccggcatgccgagcaaatgcctgcaaatcgctccccatttcacccaattgtagatatgcttaaactgggtctaacaattcgaagaatctgtagtgagccaaaccatccaaaataccagcagcgtatctcttttcggagaagtagattggttcaatttcacctagattagacaattcttcgtgatgtctattagcaactacaacagacaaagtgttacctctcatcatatcttcatcagcgcctgaaccaccagcagtaaaaacatgttctaatggaatattccattgttgcgataaccatctgacagcgtaacccttagaagctctaattggcaaaatatccaagaattgaccaaagctaatgatagtgttcacggtttgttcacctttatgtaacaattgtctaatttcttctaggtttggtgcaatagcggcgtcgtaaaagtaactgatcttgtaagcagatagttcttcctttggttgcaaagctaagcctggcaattcacctaaaattctaacaattgcatttctgttccacaaatagtcaatatgattacgccaagattgatcaggaatcaaatcaggagaggagtagatctcagtacccatagaggtgatcaacatatcaggttgtgggattctgtattctctcaaaatcttcaagacagaatccaaccttctacctgtggcaatacaaaaaccgacgttctttctatgttggtacaaaacttctaacaattcatccaaagtttgtctgtcgccaggtaaaccaccttgtaaagcacccaacaagttttgatctaaactggtaaccaaggcaccgttgtagtacaaggttcttcttctttttaagtcagaacgtttcaaaactgaagtttgttgagtcaacgcgttaatagcttcaagataagattcaacatgggatggccaagaatagtgccttttaacgccttccaaaccagattctgataagaattgccattgttgcttatcgttcaaaactttcaataacttatctgcgatatcaacttcatccaacgggttaatcaaataaccattttgacaattcttgatgatatcaacaggaccgccatcttcagtagcaacaatggggacaccacaagcagcggcttcaatcaaagtcaaaccaaaaggttcagtcaaagctggattaatgaatacaccttgggacaaagcagtaagacggaataaagcataaacgtcctcagcttggttttgcttaggataagcaaccttgccatacaaatcgtacctatcaattgttaacaacaaatcggtcaacacttcacgtggaccttgatccaaatcagtaatgtcgtcccggttaccagcaacgatgactaggttagcttgggcttgtagttgtggagattggccataagctgcaatcaacttatgaatgttctttcttggatctggacgagacaaggccaagataattggctttcttgggtgtctcaagaatctttgtaattcttgaacaattggggtttcccattcattaccttttggtgggtaaaacttttccaaatcagtacctggtggaatgacaagcatttgatctggttggtaataatcgtattgagcatattgttctgcgatttcttggtgagtagaggtaatgactctggcagctgaacctaaagtttcttcttcagcgttaatacgtctggccatattgtatctagattcaatttcatcagccttaataccagacaataatagtctagttctcttagaacgacctaaagagtgaccagtatgaactaatgggatacccaattggtgtgacaatctagtaccaacgtaaccagcatcagcgtagtgagaatgaataacatcaggcaattcaggttgttcctttaggtaatctaaagcgtgatcagcgaagttatctaagtaatcccacaacatttctttagcgatatattcttcaggaccacattcaattctaacaatttgagctctgtcaccaattaattctctaggttgtgcataatcagcatcaacttttggatccttaattaatcttgtcaaaagatcaactctagctacttgtggatttttaactagagctctagctaattccaaaacgtatttggtttgaccaccagtatcagcatctctacctaattctaagttttcacctctaatcaaaccatgaacagaaatcaacaaaatgtacttagaggagtaagacattttgtttgtttatgtgtgtttattcgaaactaagttcttggtgttttaaaactaaaaaaaagactaactataaaagtagaatttaagaagtttaagaaatagatttacagaattacaatcaatacctaccgtctttatatacttattagtcaagtaggggaataatttcagggaactggtttaaaccttttttttcagctttttccaaatcagagagagcagaaggtaatagaaggtgtaagaaaatgagatagatacatgcgtgggtcaattgccttgtgtcatcatttactccaggcaggttgcatcactccattgaggttgtgcccgttttttgcctgtttgtgccctgttctctgtagttgcgctaagagaatggacctatgaactgatggttggtgaagaaaacaatattttggtgctgggattctttttttttctggatgccagcttaaaaagcgggctccattatatttagtggatgccaggaataaacctgttcacccaagcaccatcagtgttatatattctgtgtaacccgccccctattttggcatgtacgggttacagcagaattaaaaggctaattttttgactaaataaagttaggaaaatcactactattaattatttacgtattctttgaaatggcagtattgataatgataaactcgaaaccagggcaaagcaaaataaaagaaacttaatacgttatgccgtaatgaagggctaccaaaaacgataatctcaactgtaaacaggtacaatgcggacccttttgccacaaaacatacatcattcattgccggaaaaagaaagaagtgaagacagcagtgcagccagccatgttgcgccaatctaattatagatgctggtgccctgaggatgtatctggagccagccatggcatcatgcgctaccgccggatgtaaaatccgacacgcaaaagaaaaccttcgaggttgcgcacttcgcccacccatgaaccacacggttagtccaaaaggggcagttcagattccagatgcgggaattagcttgctgccaccctcacctcactaacgctgcggtgtgcggatacttcatgctatttatagacgcgcgtgtcggaatcagcacgcgcaagaaccaaatgggaaaatcggaatgggtccagaactgctttgagtgctggctattggcgtctgatttccgttttgggaatcctttgccgcgcgcccctctcaaaactccgcacaagtcccagaaagcgggaaagaaataaaacgccaccaaaaaaaaaaataaaagccaatcctcgaagcgtgggtggtaggccctggattatcccgtacaagtatttctcaggagtaaaaaaaccgtttgttttggaattccccatttcgcggccacctacgccgctatctttgcaacaactatctgcgataactcagcaaattttgcatattcgtgttgcagtattgcgataatgggagtcttacttccaacataacggcagaaagaaatgtgagaaaattttgcatcctttgcctccgttcaagtatataaagtcggcatgcttgataatctttctttccatcctacattgttctaattattcttattctcctttattctttcctaacataccaagaaattaatcttctgtcattcgcttaaacactatatcaataatgagacaattgttgttgatttctgatttggataacacttgggtcggcgatcaacaagctttggaacatttgcaagaatacttgggtgacagaagaggtaacttttacttggcttacgctactggtagatcctaccactctgctagagaattgcaaaagcaagttggtttgatggaaccagattactggttgactgctgttggttctgaaatctatcatccagaaggtttagatcaacactgggctgattacttgtccgaacattggcaaagagatattttgcaagctattgctgatggttttgaagccttgaagccacaatctccattagaacaaaacccatggaaaatttcttatcacttagatccacaagcttgtccaaccgttattgatcaattgaccgaaatgttgaaggaaactggtattccagttcaagttattttctcctctggtaaagatgttgacttgttaccacaacgttctaataagggtaacgctactcaatacttgcaacaacatttggctatggaaccatctcaaactttggtttgtggtgactctggtaacgatattggtttgtttgaaacttctgctagaggtgttattgttagaaacgctcaaccagaattgttgcattggtacgatcaatggggtgactctagacattacagagctcaatcttctcatgctggtgctatcttggaagctattgctcattttgatttcttgtcttaagttaattcaaattaattgatatagttttttaatgagtattgaatctgtttagaaataatggaatattatttttatttatttatttatattattggtcggctcttttcttctgaaggtcaatgacaaaatgatatgaaggaaataatgatttctaaaattttacaacgtaagatatttttacaaaagcctagctcatcttttgtcatgcactattttactcacgcttgaaattaacggccagtccactgcggagtcatttcaaagtcatcctaatcgatctatcgtttttgatagctcattttggagttcgcgattgtcttctgttattcacaactgttttaatttttatttcattctggaactcttcgagttctttgtaaagtctttcatagtagcttacttgtgtccgcgtttctaaggc

SEQ ID NO: 17 - DNA, 729 bp, synthetic construct
  source 1..729: mol_type = other DNA
atgaaggttatggaatgtcaaacttacgaagaattgtctcaaatcgctgctagaattactgctgatactattaaggaaaagccagatgctgttttgggtttagctactggtggtactccagaaggtacttatagacaattgattagattacatcaaactgaaaatttgtctttccaaaatattactactgttaacttagatgaatacgctggtttgtcctctgatgatccaaactcttaccatttttacatgaatgatagatttttccaacatattgattctaagccatctagacattttattccaaacggtaacgctgatgatttggaagctgaatgtagaagatatgaacaattagttgattctttgggtgacactgatattcaattattaggtattggtagaaatggtcatattggtttcaatgaaccaggtacttccttcaaatctagaactcacgtcgttactttaaacgaacaaactagacaagctaacgctagatacttcccatctatcgattctgttcctaagaaggctttgactatgggtattcaaactattttgtctagtaagagaattttgttgttgatttctggtaaatctaaggctgaagctgttagaaagttgttggaaggtaacatttcagaagatttcccagcttctgctttgcatctacattctgatgttactgttttgattgatagagaagctgcttctttgagaccataa

SEQ ID NO: 18 - DNA, 777 bp, synthetic construct
  source 1..777: mol_type = other DNA
atgattaaggttttgttgttggatgttgatggtactttgttgtcttttgaaactcacaaggtttctcaatcttctattgacgccttgaagaaggttcatgattctggtattaagatcgtcattgctactggtagagctgcttccgatttgcatgaaattgatgctgttccatatgatggtgttattgccttgaacggtgctgaatgtgttttgagagatggttctgttattagaaaggttgctattccagctcaagattttagaaagtctatggaattagctcgtgaattcgatttcgctgttgctttagaattgaatgaaggtgtttttgttaatagattgaccccaactgttgaacaaattgctggtatcgttgaacacccagttccaccagttgttgatattgaagaaatgttcgaaagaaaagaatgttgtcaattatgtttctacttcgatgaagaagctgaacaaaaggttatgccattgttgtctggtttgtctgctactagatggcatccattgtttgctgacgttaacgttgctggtacttcaaaggctactggtttatctttgttcgctgattactatagagttaaggtttctgaaattatggcttgtggcgatggtggtaacgatattccaatgttgaaggctgctggtattggtgttgctatgggtaacgcctccgaaaaggttcaatctgttgctgatttcgttactgatactgttgataactctggtttgtacaaggctttgaagcatttcggtgttatttaa

SEQ ID NO: 19 - DNA, 3863 bp, synthetic construct
  source 1..3863: mol_type = other DNA
caacttgctctcgaagtggtcgcgaatttcttatgatttatgatttttattattaaataagttataaaaaaaataagtgtatacaaattttaaagtgactcttaggttttaaaacgaaaattcttattcttgagtaactctttcctgtaggtcaggttgctttctcaggtatagcatgaggtcgctcttattgaccacacctctaccggcatgccgagcaaatgcctgcaaatcgctccccatttcacccaattgtagatatgcttatggtctcaaagaagcagcttctctatcaatcaaaacagtaacatcagaatgtagatgcaaagcagaagctgggaaatcttctgaaatgttaccttccaacaactttctaacagcttcagccttagatttaccagaaatcaacaacaaaattctcttactagacaaaatagtttgaatacccatagtcaaagccttcttaggaacagaatcgatagatgggaagtatctagcgttagcttgtctagtttgttcgtttaaagtaacgacgtgagttctagatttgaaggaagtacctggttcattgaaaccaatatgaccatttctaccaatacctaataattgaatatcagtgtcacccaaagaatcaactaattgttcatatcttctacattcagcttccaaatcatcagcgttaccgtttggaataaaatgtctagatggcttagaatcaatatgttggaaaaatctatcattcatgtaaaaatggtaagagtttggatcatcagaggacaaaccagcgtattcatctaagttaacagtagtaatattttggaaagacaaattttcagtttgatgtaatctaatcaattgtctataagtaccttctggagtaccaccagtagctaaacccaaaacagcatctggcttttccttaatagtatcagcagtaattctagcagcgatttgagacaattcttcgtaagtttgacattccataaccttcattttgtttgtttatgtgtgtttattcgaaactaagttcttggtgttttaaaactaaaaaaaagactaactataaaagtagaatttaagaagtttaagaaatagatttacagaattacaatcaatacctaccgtctttatatacttattagtcaagtaggggaataatttcagggaactggtttaaaccttttttttcagctttttccaaatcagagagagcagaaggtaatagaaggtgtaagaaaatgagatagatacatgcgtgggtcaattgccttgtgtcatcatttactccaggcaggttgcatcactccattgaggttgtgcccgttttttgcctgtttgtgccctgttctctgtagttgcgctaagagaatggacctatgaactgatggttggtgaagaaaacaatattttggtgctgggattctttttttttctggatgccagcttaaaaagcgggctccattatatttagtggatgccaggaataaacctgttcacccaagcaccatcagtgttatatattctgtgtaacccgccccctattttggcatgtacgggttacagcagaattaaaaggctaattttttgactaaataaagttaggaaaatcactactattaattatttacgtattctttgaaatggcagtattgataatgataaactcgaaaccagggcaaagcaaaataaaagaaacttaatacgttatgccgtaatgaagggctaccaaaaacgataatctcaactgtaaacaggtacaatgcggacccttttgccacaaaacatacatcattcattgccggaaaaagaaagaagtgaagacagcagtgcagccagccatgttgcgccaatctaattatagatgctggtgccctgaggatgtatctggagccagccatggcatcatgcgctaccgccggatgtaaaatccgacacgcaaaagaaaaccttcgaggttgcgcacttcgcccacccatgaaccacacggttagtccaaaaggggcagttcagattccagatgcgggaattagcttgctgccaccctcacctcactaacgctgcggtgtgcggatacttcatgctatttatagacgcgcgtgtcggaatcagcacgcgcaagaaccaaatgggaaaatcggaatgggtccagaactgctttgagtgctggctattggcgtctgatttccgttttgggaatcctttgccgcgcgcccctctcaaaactccgcacaagtcccagaaagcgggaaagaaataaaacgccaccaaaaaaaaaaataaaagccaatcctcgaagcgtgggtggtaggccctggattatcccgtacaagtatttctcaggagtaaaaaaaccgtttgttttggaattccccatttcgcggccacctacgccgctatctttgcaacaactatctgcgataactcagcaaattttgcatattcgtgttgcagtattgcgataatgggagtcttacttccaacataacggcagaaagaaatgtgagaaaattttgcatcctttgcctccgttcaagtatataaagtcggcatgcttgataatctttctttccatcctacattgttctaattattcttattctcctttattctttcctaacataccaagaaattaatcttctgtcattcgcttaaacactatatcaataatgattaaggttttgttgttggatgttgatggtactttgttgtcttttgaaactcacaaggtttctcaatcttctattgacgccttgaagaaggttcatgattctggtattaagatcgtcattgctactggtagagctgcttccgatttgcatgaaattgatgctgttccatatgatggtgttattgccttgaacggtgctgaatgtgttttgagagatggttctgttattagaaaggttgctattccagctcaagattttagaaagtctatggaattagctcgtgaattcgatttcgctgttgctttagaattgaatgaaggtgtttttgttaatagattgaccccaactgttgaacaaattgctggtatcgttgaacacccagttccaccagttgttgatattgaagaaatgttcgaaagaaaagaatgttgtcaattatgtttctacttcgatgaagaagctgaacaaaaggttatgccattgttgtctggtttgtctgctactagatggcatccattgtttgctgacgttaacgttgctggtacttcaaaggctactggtttatctttgttcgctgattactatagagttaaggtttctgaaattatggcttgtggcgatggtggtaacgatattccaatgttgaaggctgctggtattggtgttgctatgggtaacgcctccgaaaaggttcaatctgttgctgatttcgttactgatactgttgataactctggtttgtacaaggctttgaagcatttcggtgttatttaagttaattcaaattaattgatatagttttttaatgagtattgaatctgtttagaaataatggaatattatttttatttatttatttatattattggtcggctcttttcttctgaaggtcaatgacaaaatgatatgaaggaaataatgatttctaaaattttacaacgtaagatatttttacaaaagcctagctcatcttttgtcatgcactattttactcacgcttgaaattaacggccagtccactgcggagtcatttcaaagtcatcctaatcgatctatcgtttttgatagctcattttggagttcgcgattgtcttctgttattcacaactgttttaatttttatttcattctggaactcttcgagttctttgtaaagtctttcatagtagcttactcctgcataatcggcctcac

SEQ ID NO: 20 - DNA, 3864 bp, synthetic construct
  source 1..3864: mol_type = other DNA
gcgagagccgacatacgagacgcgaatttcttatgatttatgatttttattattaaataagttataaaaaaaataagtgtatacaaattttaaagtgactcttaggttttaaaacgaaaattcttattcttgagtaactctttcctgtaggtcaggttgctttctcaggtatagcatgaggtcgctcttattgaccacacctctaccggcatgccgagcaaatgcctgcaaatcgctccccatttcacccaattgtagatatgcttatggtctcaaagaagcagcttctctatcaatcaaaacagtaacatcagaatgtagatgcaaagcagaagctgggaaatcttctgaaatgttaccttccaacaactttctaacagcttcagccttagatttaccagaaatcaacaacaaaattctcttactagacaaaatagtttgaatacccatagtcaaagccttcttaggaacagaatcgatagatgggaagtatctagcgttagcttgtctagtttgttcgtttaaagtaacgacgtgagttctagatttgaaggaagtacctggttcattgaaaccaatatgaccatttctaccaatacctaataattgaatatcagtgtcacccaaagaatcaactaattgttcatatcttctacattcagcttccaaatcatcagcgttaccgtttggaataaaatgtctagatggcttagaatcaatatgttggaaaaatctatcattcatgtaaaaatggtaagagtttggatcatcagaggacaaaccagcgtattcatctaagttaacagtagtaatattttggaaagacaaattttcagtttgatgtaatctaatcaattgtctataagtaccttctggagtaccaccagtagctaaacccaaaacagcatctggcttttccttaatagtatcagcagtaattctagcagcgatttgagacaattcttcgtaagtttgacattccataaccttcattttgtttgtttatgtgtgtttattcgaaactaagttcttggtgttttaaaactaaaaaaaagactaactataaaagtagaatttaagaagtttaagaaatagatttacagaattacaatcaatacctaccgtctttatatacttattagtcaagtaggggaataatttcagggaactggtttaaaccttttttttcagctttttccaaatcagagagagcagaaggtaatagaaggtgtaagaaaatgagatagatacatgcgtgggtcaattgccttgtgtcatcatttactccaggcaggttgcatcactccattgaggttgtgcccgttttttgcctgtttgtgccctgttctctgtagttgcgctaagagaatggacctatgaactgatggttggtgaagaaaacaatattttggtgctgggattctttttttttctggatgccagcttaaaaagcgggctccattatatttagtggatgccaggaataaacctgttcacccaagcaccatcagtgttatatattctgtgtaacccgccccctattttggcatgtacgggttacagcagaattaaaaggctaattttttgactaaataaagttaggaaaatcactactattaattatttacgtattctttgaaatggcagtattgataatgataaactcgaaaccagggcaaagcaaaataaaagaaacttaatacgttatgccgtaatgaagggctaccaaaaacgataatctcaactgtaaacaggtacaatgcggacccttttgccacaaaacatacatcattcattgccggaaaaagaaagaagtgaagacagcagtgcagccagccatgttgcgccaatctaattatagatgctggtgccctgaggatgtatctggagccagccatggcatcatgcgctaccgccggatgtaaaatccgacacgcaaaagaaaaccttcgaggttgcgcacttcgcccacccatgaaccacacggttagtccaaaaggggcagttcagattccagatgcgggaattagcttgctgccaccctcacctcactaacgctgcggtgtgcggatacttcatgctatttatagacgcgcgtgtcggaatcagcacgcgcaagaaccaaatgggaaaatcggaatgggtccagaactgctttgagtgctggctattggcgtctgatttccgttttgggaatcctttgccgcgcgcccctctcaaaactccgcacaagtcccagaaagcgggaaagaaataaaacgccaccaaaaaaaaaaataaaagccaatcctcgaagcgtgggtggtaggccctggattatcccgtacaagtatttctcaggagtaaaaaaaccgtttgttttggaattccccatttcgcggccacctacgccgctatctttgcaacaactatctgcgataactcagcaaattttgcatattcgtgttgcagtattgcgataatgggagtcttacttccaacataacggcagaaagaaatgtgagaaaattttgcatcctttgcctccgttcaagtatataaagtcggcatgcttgataatctttctttccatcctacattgttctaattattcttattctcctttattctttcctaacataccaagaaattaatcttctgtcattcgcttaaacactatatcaataatgattaaggttttgttgttggatgttgatggtactttgttgtcttttgaaactcacaaggtttctcaatcttctattgacgccttgaagaaggttcatgattctggtattaagatcgtcattgctactggtagagctgcttccgatttgcatgaaattgatgctgttccatatgatggtgttattgccttgaacggtgctgaatgtgttttgagagatggttctgttattagaaaggttgctattccagctcaagattttagaaagtctatggaattagctcgtgaattcgatttcgctgttgctttagaattgaatgaaggtgtttttgttaatagattgaccccaactgttgaacaaattgctggtatcgttgaacacccagttccaccagttgttgatattgaagaaatgttcgaaagaaaagaatgttgtcaattatgtttctacttcgatgaagaagctgaacaaaaggttatgccattgttgtctggtttgtctgctactagatggcatccattgtttgctgacgttaacgttgctggtacttcaaaggctactggtttatctttgttcgctgattactatagagttaaggtttctgaaattatggcttgtggcgatggtggtaacgatattccaatgttgaaggctgctggtattggtgttgctatgggtaacgcctccgaaaaggttcaatctgttgctgatttcgttactgatactgttgataactctggtttgtacaaggctttgaagcatttcggtgttatttaagttaattcaaattaattgatatagttttttaatgagtattgaatctgtttagaaataatggaatattatttttatttatttatttatattattggtcggctcttttcttctgaaggtcaatgacaaaatgatatgaaggaaataatgatttctaaaattttacaacgtaagatatttttacaaaagcctagctcatcttttgtcatgcactattttactcacgcttgaaattaacggccagtccactgcggagtcatttcaaagtcatcctaatcgatctatcgtttttgatagctcattttggagttcgcgattgtcttctgttattcacaactgttttaatttttatttcattctggaactcttcgagttctttgtaaagtctttcatagtagcttacttgtgtccgcgtttctaaggc

SEQ ID NO: 21 - DNA, 3865 bp, synthetic construct
  source 1..3865: mol_type = other DNA
accggtttgaatttattgtcacgcgaatttcttatgatttatgatttttattattaaataagttataaaaaaaataagtgtatacaaattttaaagtgactcttaggttttaaaacgaaaattcttattcttgagtaactctttcctgtaggtcaggttgctttctcaggtatagcatgaggtcgctcttattgaccacacctctaccggcatgccgagcaaatgcctgcaaatcgctccccatttcacccaattgtagatatgcttatggtctcaaagaagcagcttctctatcaatcaaaacagtaacatcagaatgtagatgcaaagcagaagctgggaaatcttctgaaatgttaccttccaacaactttctaacagcttcagccttagatttaccagaaatcaacaacaaaattctcttactagacaaaatagtttgaatacccatagtcaaagccttcttaggaacagaatcgatagatgggaagtatctagcgttagcttgtctagtttgttcgtttaaagtaacgacgtgagttctagatttgaaggaagtacctggttcattgaaaccaatatgaccatttctaccaatacctaataattgaatatcagtgtcacccaaagaatcaactaattgttcatatcttctacattcagcttccaaatcatcagcgttaccgtttggaataaaatgtctagatggcttagaatcaatatgttggaaaaatctatcattcatgtaaaaatggtaagagtttggatcatcagaggacaaaccagcgtattcatctaagttaacagtagtaatattttggaaagacaaattttcagtttgatgtaatctaatcaattgtctataagtaccttctggagtaccaccagtagctaaacccaaaacagcatctggcttttccttaatagtatcagcagtaattctagcagcgatttgagacaattcttcgtaagtttgacattccataaccttcattttgtttgtttatgtgtgtttattcgaaactaagttcttggtgttttaaaactaaaaaaaagactaactataaaagtagaatttaagaagtttaagaaatagatttacagaattacaatcaatacctaccgtctttatatacttattagtcaagtaggggaataatttcagggaactggtttaaaccttttttttcagctttttccaaatcagagagagcagaaggtaatagaaggtgtaagaaaatgagatagatacatgcgtgggtcaattgccttgtgtcatcatttactccaggcaggttgcatcactccattgaggttgtgcccgttttttgcctgtttgtgccctgttctctgtagttgcgctaagagaatggacctatgaactgatggttggtgaagaaaacaatattttggtgctgggattctttttttttctggatgccagcttaaaaagcgggctccattatatttagtggatgccaggaataaacctgttcacccaagcaccatcagtgttatatattctgtgtaacccgccccctattttggcatgtacgggttacagcagaattaaaaggctaattttttgactaaataaagttaggaaaatcactactattaattatttacgtattctttgaaatggcagtattgataatgataaactcgaaaccagggcaaagcaaaataaaagaaacttaatacgttatgccgtaatgaagggctaccaaaaacgataatctcaactgtaaacaggtacaatgcggacccttttgccacaaaacatacatcattcattgccggaaaaagaaagaagtgaagacagcagtgcagccagccatgttgcgccaatctaattatagatgctggtgccctgaggatgtatctggagccagccatggcatcatgcgctaccgccggatgtaaaatccgacacgcaaaagaaaaccttcgaggttgcgcacttcgcccacccatgaaccacacggttagtccaaaaggggcagttcagattccagatgcgggaattagcttgctgccaccctcacctcactaacgctgcggtgtgcggatacttcatgctatttatagacgcgcgtgtcggaatcagcacgcgcaagaaccaaatgggaaaatcggaatgggtccagaactgctttgagtgctggctattggcgtctgatttccgttttgggaatcctttgccgcgcgcccctctcaaaactccgcacaagtcccagaaagcgggaaagaaataaaacgccaccaaaaaaaaaaataaaagccaatcctcgaagcgtgggtggtaggccctggattatcccgtacaagtatttctcaggagtaaaaaaaccgtttgttttggaattccccatttcgcggccacctacgccgctatctttgcaacaactatctgcgataactcagcaaattttgcatattcgtgttgcagtattgcgataatgggagtcttacttccaacataacggcagaaagaaatgtgagaaaattttgcatcctttgcctccgttcaagtatataaagtcggcatgcttgataatctttctttccatcctacattgttctaattattcttattctcctttattctttcctaacataccaagaaattaatcttctgtcattcgcttaaacactatatcaataatgattaaggttttgttgttggatgttgatggtactttgttgtcttttgaaactcacaaggtttctcaatcttctattgacgccttgaagaaggttcatgattctggtattaagatcgtcattgctactggtagagctgcttccgatttgcatgaaattgatgctgttccatatgatggtgttattgccttgaacggtgctgaatgtgttttgagagatggttctgttattagaaaggttgctattccagctcaagattttagaaagtctatggaattagctcgtgaattcgatttcgctgttgctttagaattgaatgaaggtgtttttgttaatagattgaccccaactgttgaacaaattgctggtatcgttgaacacccagttccaccagttgttgatattgaagaaatgttcgaaagaaaagaatgttgtcaattatgtttctacttcgatgaagaagctgaacaaaaggttatgccattgttgtctggtttgtctgctactagatggcatccattgtttgctgacgttaacgttgctggtacttcaaaggctactggtttatctttgttcgctgattactatagagttaaggtttctgaaattatggcttgtggcgatggtggtaacgatattccaatgttgaaggctgctggtattggtgttgctatgggtaacgcctccgaaaaggttcaatctgttgctgatttcgttactgatactgttgataactctggtttgtacaaggctttgaagcatttcggtgttatttaagttaattcaaattaattgatatagttttttaatgagtattgaatctgtttagaaataatggaatattatttttatttatttatttatattattggtcggctcttttcttctgaaggtcaatgacaaaatgatatgaaggaaataatgatttctaaaattttacaacgtaagatatttttacaaaagcctagctcatcttttgtcatgcactattttactcacgcttgaaattaacggccagtccactgcggagtcatttcaaagtcatcctaatcgatctatcgtttttgatagctcattttggagttcgcgattgtcttctgttattcacaactgttttaatttttatttcattctggaactcttcgagttctttgtaaagtctttcatagtagcttactcaactcagaagtttgacagc

SEQ ID NO: 22 - DNA, 2215 bp, synthetic construct
  source 1..2215: mol_type = other DNA
cggaataccaagcccattgaaccagggcaaagcaaaataaaagaaacttaatacgttatgccgtaatgaagggctaccaaaaacgataatctcaactgtaaacaggtacaatgcggacccttttgccacaaaacatacatcattcattgccggaaaaagaaagaagtgaagacagcagtgcagccagccatgttgcgccaatctaattatagatgctggtgccctgaggatgtatctggagccagccatggcatcatgcgctaccgccggatgtaaaatccgacacgcaaaagaaaaccttcgaggttgcgcacttcgcccacccatgaaccacacggttagtccaaaaggggcagttcagattccagatgcgggaattagcttgctgccaccctcacctcactaacgctgcggtgtgcggatacttcatgctatttatagacgcgcgtgtcggaatcagcacgcgcaagaaccaaatgggaaaatcggaatgggtccagaactgctttgagtgctggctattggcgtctgatttccgttttgggaatcctttgccgcgcgcccctctcaaaactccgcacaagtcccagaaagcgggaaagaaataaaacgccaccaaaaaaaaaaataaaagccaatcctcgaagcgtgggtggtaggccctggattatcccgtacaagtatttctcaggagtaaaaaaaccgtttgttttggaattccccatttcgcggccacctacgccgctatctttgcaacaactatctgcgataactcagcaaattttgcatattcgtgttgcagtattgcgataatgggagtcttacttccaacataacggcagaaagaaatgtgagaaaattttgcatcctttgcctccgttcaagtatataaagtcggcatgcttgataatctttctttccatcctacattgttctaattattcttattctcctttattctttcctaacataccaagaaattaatcttctgtcattcgcttaaacactatatcaataatgattaaggttttgttgttggatgttgatggtactttgttgtcttttgaaactcacaaggtttctcaatcttctattgacgccttgaagaaggttcatgattctggtattaagatcgtcattgctactggtagagctgcttccgatttgcatgaaattgatgctgttccatatgatggtgttattgccttgaacggtgctgaatgtgttttgagagatggttctgttattagaaaggttgctattccagctcaagattttagaaagtctatggaattagctcgtgaattcgatttcgctgttgctttagaattgaatgaaggtgtttttgttaatagattgaccccaactgttgaacaaattgctggtatcgttgaacacccagttccaccagttgttgatattgaagaaatgttcgaaagaaaagaatgttgtcaattatgtttctacttcgatgaagaagctgaacaaaaggttatgccattgttgtctggtttgtctgctactagatggcatccattgtttgctgacgttaacgttgctggtacttcaaaggctactggtttatctttgttcgctgattactatagagttaaggtttctgaaattatggcttgtggcgatggtggtaacgatattccaatgttgaaggctgctggtattggtgttgctatgggtaacgcctccgaaaaggttcaatctgttgctgatttcgttactgatactgttgataactctggtttgtacaaggctttgaagcatttcggtgttatttaagttaattcaaattaattgatatagttttttaatgagtattgaatctgtttagaaataatggaatattatttttatttatttatttatattattggtcggctcttttcttctgaaggtcaatgacaaaatgatatgaaggaaataatgatttctaaaattttacaacgtaagatatttttacaaaagcctagctcatcttttgtcatgcactattttactcacgcttgaaattaacggccagtccactgcggagtcatttcaaagtcatcctaatcgatctatcgtttttgatagctcattttggagttcgcgattgtcttctgttattcacaactgttttaatttttatttcattctggaactcttcgagttctttgtaaagtctttcatagtagcttacttttcttggcattggcaaatc

SEQ ID NO: 23 - DNA, 804 bp, synthetic construct
  source 1..804: mol_type = other DNA
atgcaccctatgcttaacatagcggttagggccgctagaaaggctggtaatttgattgctaagaactacgaaaccccagatgctgttgaagcttctcaaaagggttccaacgatttcgttactaacgttgataaagctgctgaagccgttattatcgatactattagaaagtcttacccacaacatactatcattactgaagaatctggtgaattggaaggtactgatcaagatgttcaatgggttattgatccattggatggtactactaactttattaagagattgccacatttcgccgtttctattgctgttagaattaagggtagaaccgaagtcgctgttgtttacgatcctatgcgtaacgaattgttcactgctactagaggtcaaggtgctcaattgaacggttatagattaagaggttctactgctagagacttagatggtaccattttagctactggtttccctttcaaggctaagcaatacgctactacttacatcaacattgttggtaaattgttcaacgaatgtgctgatttcagacgtactggttccgctgctttggatttggcttacgttgctgctggtagagttgacggtttctttgaaattggtttgagaccatgggatttcgctgctggtgaattgttggttagagaagctggtggtattgtttccgattttactggtggtcataactatatgttgaccggtaatatcgttgctggtaatccaagagttgttaaggctatgttggctaacatgagagatgaattgtctgatgctttgaagagataa

SEQ ID NO: 24 - DNA, 2710 bp, synthetic construct
  source 1..2710: mol_type = other DNA
taactcttcgtatgaggattttcgatggagcaggatgaggagaaatagtaccacatgtatatatccattacaaaaaggtttatatacaattacaatagacccttgttggggtttctgaaaaaagaagtagtcgatgccatcggcaataatacggaattacgagaaacacaatcccgatccttttttgggtaattacttcaccgattctaccgatttatcatgccaaaaaaaattcaccgtgggttctagaagtgccctttgaggattgtagccactctaacccacacggcctccttactagctgactaaggtgacaaaaccgcaaggactggaaagtcgccactcatctgaaaattctcaagtttttcactactgagtttatgctttcgaatttttttgttcggtaatagcacggcggttcgattcaattccgccgctccgagcgatgctccgcaaaactcagtaataagctttctgatggttcaccccttttttagcacgcggggtgtaactcaacagaaaaatgtgccatagaagggtaccggccgcaaattaaagccttcgagcgtcccaaaaccttctcaagcaaggttttcagtataatgttacatgcgtacacgcgtctgtacagaaaaaaaagaaaaatttgaaatataaataacgttcttaatactaacataactataaaaaaataaatagggacctagacttcaggttgtctaactccttccttttcggttagagcggatgtggggggagggcgtgaatgtaagcgtgacataactaattacatgactcgaggtcgacggtatcttatctcttcaaagcatcagacaattcatctctcatgttagccaacatagccttaacaactcttggattaccagcaacgatattaccggtcaacatatagttatgaccaccagtaaaatcggaaacaataccaccagcttctctaaccaacaattcaccagcagcgaaatcccatggtctcaaaccaatttcaaagaaaccgtcaactctaccagcagcaacgtaagccaaatccaaagcagcggaaccagtacgtctgaaatcagcacattcgttgaacaatttaccaacaatgttgatgtaagtagtagcgtattgcttagccttgaaagggaaaccagtagctaaaatggtaccatctaagtctctagcagtagaacctcttaatctataaccgttcaattgagcaccttgacctctagtagcagtgaacaattcgttacgcataggatcgtaaacaacagcgacttcggttctacccttaattctaacagcaatagaaacggcgaaatgtggcaatctcttaataaagttagtagtaccatccaatggatcaataacccattgaacatcttgatcagtaccttccaattcaccagattcttcagtaatgatagtatgttgtgggtaagactttctaatagtatcgataataacggcttcagcagctttatcaacgttagtaacgaaatcgttggaacccttttgagaagcttcaacagcatctggggtttcgtagttcttagcaatcaaattaccagcctttctagcggccctaaccgctatgttaagcatagggtgcatcattttgtttgtttatgtgtgtttattcgaaactaagttcttggtgttttaaaactaaaaaaaagactaactataaaagtagaatttaagaagtttaagaaatagatttacagaattacaatcaatacctaccgtctttatatacttattagtcaagtaggggaataatttcagggaactggtttaaaccttttttttcagctttttccaaatcagagagagcagaaggtaatagaaggtgtaagaaaatgagatagatacatgcgtgggtcaattgccttgtgtcatcatttactccaggcaggttgcatcactccattgaggttgtgcccgttttttgcctgtttgtgccctgttctctgtagttgcgctaagagaatggacctatgaactgatggttggtgaagaaaacaatattttggtgctgggattctttttttttctggatgccagcttaaaaagcgggctccattatatttagtggatgccaggaataaacctgttcacccaagcaccatcagtgttatatattctgtgtaacccgccccctattttggcatgtacgggttacagcagaattaaaaggctaattttttgactaaataaagttaggaaaatcactactattaattatttacgtattctttgaaatggcagtattgataatgataaactcgaatagcttcaaaatgtttctactccttttttactcttccagattttctcggactccgcgcatcgccgtaccacttcaaaacacccaagcacagcatactaaatttcccctctttcttcctctagggtgtcgttaattacccgtactaaaggtttggaaaagaaaaaagagaccgcctcgtttctttttcttcgtcgaaaaaggcaataaaaatttttatcacgtttctttttcttgaaaatttttttttttgatttttttctctttcgatgacctcccattgatatttaagttaataaacggtcttcaatttctcaagtttcagtttcatttttcttgttctattacaactttttttacttcttgctcattagaaagaaagcatagcaatctaatctaagttttaattacaaaatg

SEQ ID NO: 25 - DNA, 4420 bp, synthetic construct
  source 1..4420: mol_type = other DNA
atagcttcaaaatgtttctactccttttttactcttccagattttctcggactccgcgcatcgccgtaccacttcaaaacacccaagcacagcatactaaatttcccctctttcttcctctagggtgtcgttaattacccgtactaaaggtttggaaaagaaaaaagagaccgcctcgtttctttttcttcgtcgaaaaaggcaataaaaatttttatcacgtttctttttcttgaaaatttttttttttgatttttttctctttcgatgacctcccattgatatttaagttaataaacggtcttcaatttctcaagtttcagtttcatttttcttgttctattacaactttttttacttcttgctcattagaaagaaagcatagcaatctaatctaagttttaattacaaaatgatgctttttgataacaaaaatcgcggtgctttaaactcactgaacacaccagatattgcttctttatcaatatcatccatgtcggactatcacgtgtttgattttcccggtaaggacctgcagagagaggaagtgatagatttgctagatcagcaagggtttattcccgacgatttgatcgaacaagaagtagattggttttataactcattgggtattgacgatttgttcttctcgagagaatctccccaattaatctcgaatatcatacattctttgtatgcttcaaagctagatttctttgcgaagtccaaattcaacggaattcagccaaggctattcagcattaaaaacaaaattataactaatgataatcatgccatctttatggaatctaatactggtgtcagcataagcgattctcagcaaaaaaactttaaatttgctagtgacgccgtcggaaacgatactttggagcatggtaaggataccatcaaaaaaaataggattgaaatggatgattcttgtccaccttatgaattagattccgaaattgatgaccttttcctggataacaagtctcaaaaaaactgcagattagtttctttttgggctccagaaagcgaattaaagctaacttttgtttatgagagtgtttaccctaatgatgatccagccggcgtagatatttcctctcaggatttgctgaaaggtgatattgaatcgattagtgataagaccatgtacaaagtttcgtcgaacgaaaataaaaaactatacggtctcttacttaagttggttaaagaaagagaaggtcctgtcattaagactactcgctccgtagaaaataaggatgaaattaggttattagtcgcttacaagcgattcaccactaagcgttattactctgctttgaactctttgttccactattacaagttgaaaccttctaagttctatttagagtcgtttaatgttaaggatgatgacatcattatcttttccgtttatttgaacgagaaccagcaattggaagatgttctacttcacgatgtggaggcagcattgaaacaggttgaaagagaagcttcattgctatacgctatcccaaacaattctttccatgaggtttaccagagacgtcaattctcgcccaaagaagctatatatgctcatattggtgctatattcattaaccattttgttaatcgtttaggctctgattatcaaaaccttttatctcaaatcaccattaagcgtaatgatactactcttttggagattgtagaaaacctaaaaagaaagttaagaaatgaaaccttaactcagcaaactattatcaacatcatgtcgaagcattacactataatttccaagttgtataaaaattttgctcaaattcactattatcataatagtactaaagatatggagaagacattatcttttcaaagactggaaaaagtggagccttttaagaatgaccaagagttcgaagcttacttgaataaattcattccaaatgattcacctgatttgttgatcctgaaaacactgaacatcttcaacaagtctattttgaagacaaatttctttattacaagaaaagtagcaatatcattcagattagatccttccctggtgatgacaaaattcgaatatccagagacaccctatggtatattttttgtcgttggtaatactttcaaagggttccatatcaggttcagagatatcgcaaggggcggtattcgtatagtctgttccaggaatcaggatatttatgatttgaattccaagaacgttattgatgagaactatcaattggcctctactcagcaacgtaaaaataaggatattccagagggtggctctaaaggtgtcatcttattgaacccaggattggtagaacatgaccagacatttgtcgccttttcccaatatgtggatgcaatgattgacattctaatcaacgatccattaaaggaaaactatgtcaaccttttaccaaaggaggaaatattattttttggcccagatgaaggaactgctggtttcgtggattgggcaactaaccatgctcgtgtgaggaactgcccatggtggaaatcatttttgactggaaaatccccatctttgggtggtattccccatgacgaatatggtatgacttctctgggtgttcgtgcttatgttaataaaatttacgaaactttaaacttgacaaattctactgtttacaaattccaaactggtggtccggatggtgatttgggatccaatgaaattcttttatcttcgccaaacgaatgttatttggcaattctggacggttcaggtgtcctgtgtgatcctaaaggtttagataaagatgaattatgccgcttggcacatgaaaggaaaatgatttccgatttcgacacttccaaattatcaaacaacggattttttgtttctgtggatgcaatggatatcatgctaccaaatggtacaattgtagctaacggcacaaccttcagaaacacctttcatactcaaattttcaaatttgtggatcatgtcgacatttttgttccatgcggtggtagaccaaactcaattactctaaataatctacattattttgttgacgaaaagactgggaaatgtaaaattccatatattgtggagggtgccaatctatttataacgcaacctgctaaaaatgctttggaggaacatggctgtattctgttcaaagatgcttctgcaaacaaaggtggtgtcacatcttcatcaatggaagtgttggcctcactagcgcttaacgataacgacttcgtgcacaaatttattggagatgttagtggtgagaggtctgcgttgtacaagtcgtacgttgtagaagtgcagtcaagaattcagaaaaatgctgaattagagtttggtcagttatggaatttgaatcaactaaatggaacccacatttcagaaatttcaaaccaattgtccttcactataaacaaattgaacgacgatctagttgcttctcaagagttgtggctcaatgatctaaaattaagaaactacctattgttggataaaataattccaaaaattctgattgatgttgctgggcctcagtccgtattggaaaacattccagagagctatttgaaagttcttctgtcgagttacttatcaagcacttttgtttaccagaacggtatcgatgttaacattggaaaattcttggaatttattggtgggttaaaaagagaagcggaggcaagtgcttgagcgaatttcttatgatttatgatttttattattaaataagttataaaaaaaataagtgtatacaaattttaaagtgactcttaggttttaaaacgaaaattcttattcttgagtaactctttcctgtaggtcaggttgctttctcaggtatagcatgaggtcgctcttattgaccacacctctaccggcatgccgagcaaatgcctgcaaatcgctccccatttcacccaattgtagatatgcccacaagtaaagctcgttgaccagttgatcagttgaggggggtacacacgactagcgctttcagatattaaaaagtttagatgtaggttttagcggtaacagttatataaatcgtgtttcttctcttgatgaaacaaaaaaatgctagaaaaactttgtcgtttcttacttttggtgcgctttgcagttttcgtggctagacttagaatcatttctcctcagatttcttgattaaagtttggtgcgaagccctactctaacattggtgttcttcttttcattcacgcaagttaagtccaggaaggtgagcaaatgctcatccttctgttcatgcgtgacggctgaattatccttatctggcgtacccgtgcagccgtttccgtgcctcggttcctccgagatatccttagggaccgccagggaccatgattgcgtcaactgttgtcaccgctccagaggatcctctgtaaccttttcaaccat

SEQ ID NO: 26 - DNA, 1602 bp, synthetic construct
  source 1..1602: mol_type = other DNA
atgacagaagataatattgctccaatcacctccgttaaagtagttaccgacaagtgcacgtacaaggacaacgagctgctcaccaagtacagctacgaaaatgctgtagttacgaagacagctagtggccgcttcgatgtcacgcccactgttcaagactacgtgttcaaacttgacttaaaaaagccggaaaaactaggaattatgctcattgggttaggtggcaacaatggctccactttagtggcctcggtattggcgaataagcacaatgtggagtttcaaactaaggaaggcgttaagcaaccaaactacttcggctccatgactcaatgttctaccttgaaactgggtatcgatgcggaggggaatgacgtttatgctccttttaactctctgttgcccatggttagcccaaacgactttgtcgtctctggttgggacatcaataacgcagatctatacgaagctatgcagagaagtcaagttctcgaatatgatctgcaacaacgcttgaaggcgaagatgtccttggtgaagcctcttccttccatttactaccctgatttcattgcagctaatcaagatgagagagccaataactgcatcaatttggatgaaaaaggcaacgtaaccacgaggggtaagtggacccatctgcaacgcatcagacgcgatatccagaatttcaaagaagaaaacgcccttgataaagtaatcgttctttggactgcaaatactgagaggtacgtagaagtatctcctggtgttaatgacaccatggaaaacctcttgcagtctattaagaatgaccatgaagagattgctccttccacgatctttgcagcagcatctatcttggaaggtgtcccctatattaatggttcaccgcagaatacttttgttcccggcttggttcagctggctgagcatgagggtacattcattgcgggagacgatctcaagtcgggacaaaccaagttgaagtctgttctggcccagttcttagtggatgcaggtattaaaccggtctccattgcatcctataaccatttaggcaataatgacggttataacttatctgctccaaaacaatttaggtctaaggagatttccaaaagttctgtcatagatgacatcatcgcgtctaatgatatcttgtacaatgataaactgggtaaaaaagttgaccactgcattgtcatcaaatatatgaagcccgtcggggactcaaaagtggcaatggacgagtattacagtgagttgatgttaggtggccataaccggatttccattcacaatgtttgcgaagattctttactggctacgcccttgatcatcgatcttttagtcatgactgagttttgtacaagagtgtcctataagaaggtggacccagttaaagaagatgctggcaaatttgagaacttttatccagttttaaccttcttgagttactggttaaaagctccattaacaagaccaggatttcacccggtgaatggcttaaacaagcaaagaaccgccttagaaaattttttaagattgttgattggattgccttctcaaaacgaactaagattcgaagagagattgttgtaa

SEQ ID NO: 27 - DNA, 1755 bp, synthetic construct
  source 1..1755: mol_type = other DNA
atgggaatacacataccatatctcacgtcaaagacatcgcaatcaaatgttggtgatgccgttggcaacgctgatagtgtagagttcaacagtgagcatgactcaccttcaaagagaggtaaaattacacttgagtcacatgaaatacagagggctcccgctagcgatgatgaagataggattcaaattaaacccgtgaacgacgaggatgacacgtcggtcatgatcacttttaaccaatctctttcgcccttcatcatcactctgacttttgtcgcatccatatccggtttcatgtttggttacgacactggttatatatccagtgcgctgatctcgatcggcacagatctggaccacaaggtacttacttatggggagaaggaaattgtcactgcggctacctctctgggagctttgattaccagtattttcgccggtactgcagctgacatatttggtaggaaacgttgtttaatgggttcgaatctgatgtttgtcattggcgcaatcttacaggtctccgcacacacattctggcaaatggctgttggtagactgatcatgggtttcggtgtcggtatcggctccttgatcgcgccacttttcatcagtgaaattgctcccaaaatgatcagagggagactaactgtcatcaattccttatggttgactggtggtcaattagtcgcttacggttgcggtgctgggttaaactacgtcaacaatggttggagaattcttgttggattgtcactaattcccactgctgtgcaattcacatgcctgtgctttttacctgacactccaagatactacgttatgaagggcgacttggcaagggctactgaggtgttgaagagaagttacactgacacttcggaggaaatcattgaacgtaaggtggaagaacttgttactttgaatcaatctattcctggtaagaatgtccctgaaaaagtctggaataccatcaaagaattgcacacagtaccatctaatctaagggctttgatcattggttgtggtttacaagcaattcaacagtttaccggttggaattcgttgatgtatttctctggtaccatcttcgaaactgtcggtttcaaaaattcttccgctgtttcaatcatcgtgtccggtaccaattttattttcactttagttgcctttttttccattgacaaaataggccgtagaaccatattattgattggattaccaggcatgaccatggctttagtcgtgtgctctattgctttccattttctaggtattaagtttgatggcgctgtcgctgtggtggtttcctccggtttctcctcttggggtattgtgatcatcgtatttattatcgtatttgctgcgttctacgctcttggtatcggtactgttccatggcaacaatcggaactattcccccaaaacgtgagaggtattgggacttcatatgcaactgctacaaactgggctggttcactggttattgcatccacatttttgaccatgttacagaatatcactcctgcaggtacatttgcctttttcgcgggattgtcgtgcttatcaaccattttctgctacttctgttatccagaattatcgggattggagttagaagaggtacaaactattttgaaggacgggttcaacatcaaagcctcgaaagctttggccaagaagagaaaacagcaagttgccagagttcatgaattgaaatatgaaccaactcaagagattatagaggatatatag

SEQ ID NO: 28 - DNA, 4276 bp, synthetic construct
  source 1..4276: mol_type = other DNA
tgtgccccttaaaattcatatacactttatgtttaattcgacaggtataacagaaagaaacaaggaaaacaatgcaattaatcattaactgcaccaacttttatatgaatatattgtgctacatgtcttaattagtcctctgtgaatgagcatcacaaagaatcacgaggaaaagattgattacttaatattgataggaatcagccgcggaaatggaaatcttggtaatataattttaatgcggcacgctgaaaattgatggcggcctgctaggagccctattgattccgcggaaataggcggattattacaaacgttgagcattcagcaggtgcggctgtgccttttcactttcagctaagatgtttgcaagcaagaattaacagataagccgcttcgctagtaacgcaactcattgtgtttttaatggaagctaaggatggttgaaattatgggtaccctgagataagattattaactatgatgtaagtattaatcattataataaggggtacctgctcattcgcatttatgtacccatgtataaccttccaagttagttcttgggaaacgaaaattatattgaattttttattgaatttttagcgtatcctttcgccatcctgataatcatgataaccttgagggaagattatcttgcgatgggagggatcaaatttagcaaattttgactctatgtcaatctcgtttccaaaaatgcaacacctcatcgttatgacgacaattggagacaaaaaggttaacaataacataatactctttttatagaataccttataaaatgtatgttatttaagtaacttataaatctttatttgagttgaaaagaaaaaccatgtctttatataaaatttaaaaaatataattcaaaaaaataatatcttcattcaatcatgattctttttttacaacaatctctcttcgaatcttagttcgttttgagaaggcaatccaatcaacaatcttaaaaaattttctaaggcggttctttgcttgtttaagccattcaccgggtgaaatcctggtcttgttaatggagcttttaaccagtaactcaagaaggttaaaactggataaaagttctcaaatttgccagcatcttctttaactgggtccaccttcttataggacactcttgtacaaaactcagtcatgactaaaagatcgatgatcaagggcgtagccagtaaagaatcttcgcaaacattgtgaatggaaatccggttatggccacctaacatcaactcactgtaatactcgtccattgccacttttgagtccccgacgggcttcatatatttgatgacaatgcagtggtcaacttttttacccagtttatcattgtacaagatatcattagacgcgatgatgtcatctatgacagaacttttggaaatctccttagacctaaattgttttggagcagataagttataaccgtcattattgcctaaatggttataggatgcaatggagaccggtttaatacctgcatccactaagaactgggccagaacagacttcaacttggtttgtcccgacttgagatcgtctcccgcaatgaatgtaccctcatgctcagccagctgaaccaagccgggaacaaaagtattctgcggtgaaccattaatataggggacaccttccaagatagatgctgctgcaaagatcgtggaaggagcaatctcttcatggtcattcttaatagactgcaagaggttttccatggtgtcattaacaccaggagatacttctacgtacctctcagtatttgcagtccaaagaacgattactttatcaagggcgttttcttctttgaaattctggatatcgcgtctgatgcgttgcagatgggtccacttacccctcgtggttacgttgcctttttcatccaaattgatgcagttattggctctctcatcttgattagctgcaatgaaatcagggtagtaaatggaaggaagaggcttcaccaaggacatcttcgccttcaagcgttgttgcagatcatattcgagaacttgacttctctgcatagcttcgtatagatctgcgttattgatgtcccaaccagagacgacaaagtcgtttgggctaaccatgggcaacagagagttaaaaggagcataaacgtcattcccctccgcatcgatacccagtttcaaggtagaacattgagtcatggagccgaagtagtttggttgcttaacgccttccttagtttgaaactccacattgtgcttattcgccaataccgaggccactaaagtggagccattgttgccacctaacccaatgagcataattcctagtttttccggcttttttaagtcaagtttgaacacgtagtcttgaacagtgggcgtgacatcgaagcggccactagctgtcttcgtaactacagcattttcgtagctgtacttggtgagcagctcgttgtccttgtacgtgcacttgtcggtaactactttaacggaggtgattggagcaatattatcttctgtcattttgttatatttgttgtaaaaagtagataattacttccttgatgatctgtaaaaaagagaaaaagaaagcatctaagaacttgaaaaactacgaattagaaaagaccaaatatgtatttcttgcattgaccaatttatgcaagtttatatatatgtaaatgtaagtttcacgaggttctactaaactaaaccacccccttggttagaagaaaagagtgtgtgagaacaggctgttgttgtcacacgattcggacaattctgtttgaaagagagagagtaacagtacgatcgaacgaactttgctctggagatcacagtgggcatcatagcatgtggtactaaaccctttcccgccattccagaaccttcgattgcttgttacaaaacctgtgagccgtcgctaggaccttgttgtgtgacgaaattggaagctgcaatcaataggaagacaggaagtcgagcgtgtctgggttttttcagttttgttctttttgcaaacaaatcacgagcgacggtaatttctttctcgataagaggccacgtgctttatgagggtaacatcaattcaagaaggagggaaacacttcctttttctggccctgataatagtatgagggtgaagccaaaataaaggattcgcgcccaaatcggcatctttaaatgcaggtatgcgatagttcctcactctttccttactcacgagtaattcttgcaaatgcctattgtgcagatgttataatatctgtgcgtaaccagggcaaagcaaaataaaagaaacttaatacgttatgccgtaatgaagggctaccaaaaacgataatctcaactgtaaacaggtacaatgcggacccttttgccacaaaacatacatcattcattgccggaaaaagaaagaagtgaagacagcagtgcagccagccatgttgcgccaatctaattatagatgctggtgccctgaggatgtatctggagccagccatggcatcatgcgctaccgccggatgtaaaatccgacacgcaaaagaaaaccttcgaggttgcgcacttcgcccacccatgaaccacacggttagtccaaaaggggcagttcagattccagatgcgggaattagcttgctgccaccctcacctcactaacgctgcggtgtgcggatacttcatgctatttatagacgcgcgtgtcggaatcagcacgcgcaagaaccaaatgggaaaatcggaatgggtccagaactgctttgagtgctggctattggcgtctgatttccgttttgggaatcctttgccgcgcgcccctctcaaaactccgcacaagtcccagaaagcgggaaagaaataaaacgccaccaaaaaaaaaaataaaagccaatcctcgaagcgtgggtggtaggccctggattatcccgtacaagtatttctcaggagtaaaaaaaccgtttgttttggaattccccatttcgcggccacctacgccgctatctttgcaacaactatctgcgataactcagcaaattttgcatattcgtgttgcagtattgcgataatgggagtcttacttccaacataacggcagaaagaaatgtgagaaaattttgcatcctttgcctccgttcaagtatataaagtcggcatgcttgataatctttctttccatcctacattgttctaattattcttattctcctttattctttcctaacataccaagaaattaatcttctgtcattcgcttaaacactatatcaata

SEQ ID NO: 29 - DNA, 3678 bp, synthetic construct
  source 1..3678: mol_type = other DNA
aaccagggcaaagcaaaataaaagaaacttaatacgttatgccgtaatgaagggctaccaaaaacgataatctcaactgtaaacaggtacaatgcggacccttttgccacaaaacatacatcattcattgccggaaaaagaaagaagtgaagacagcagtgcagccagccatgttgcgccaatctaattatagatgctggtgccctgaggatgtatctggagccagccatggcatcatgcgctaccgccggatgtaaaatccgacacgcaaaagaaaaccttcgaggttgcgcacttcgcccacccatgaaccacacggttagtccaaaaggggcagttcagattccagatgcgggaattagcttgctgccaccctcacctcactaacgctgcggtgtgcggatacttcatgctatttatagacgcgcgtgtcggaatcagcacgcgcaagaaccaaatgggaaaatcggaatgggtccagaactgctttgagtgctggctattggcgtctgatttccgttttgggaatcctttgccgcgcgcccctctcaaaactccgcacaagtcccagaaagcgggaaagaaataaaacgccaccaaaaaaaaaaataaaagccaatcctcgaagcgtgggtggtaggccctggattatcccgtacaagtatttctcaggagtaaaaaaaccgtttgttttggaattccccatttcgcggccacctacgccgctatctttgcaacaactatctgcgataactcagcaaattttgcatattcgtgttgcagtattgcgataatgggagtcttacttccaacataacggcagaaagaaatgtgagaaaattttgcatcctttgcctccgttcaagtatataaagtcggcatgcttgataatctttctttccatcctacattgttctaattattcttattctcctttattctttcctaacataccaagaaattaatcttctgtcattcgcttaaacactatatcaataatgggaatacacataccatatctcacgtcaaagacatcgcaatcaaatgttggtgatgccgttggcaacgctgatagtgtagagttcaacagtgagcatgactcaccttcaaagagaggtaaaattacacttgagtcacatgaaatacagagggctcccgctagcgatgatgaagataggattcaaattaaacccgtgaacgacgaggatgacacgtcggtcatgatcacttttaaccaatctctttcgcccttcatcatcactctgacttttgtcgcatccatatccggtttcatgtttggttacgacactggttatatatccagtgcgctgatctcgatcggcacagatctggaccacaaggtacttacttatggggagaaggaaattgtcactgcggctacctctctgggagctttgattaccagtattttcgccggtactgcagctgacatatttggtaggaaacgttgtttaatgggttcgaatctgatgtttgtcattggcgcaatcttacaggtctccgcacacacattctggcaaatggctgttggtagactgatcatgggtttcggtgtcggtatcggctccttgatcgcgccacttttcatcagtgaaattgctcccaaaatgatcagagggagactaactgtcatcaattccttatggttgactggtggtcaattagtcgcttacggttgcggtgctgggttaaactacgtcaacaatggttggagaattcttgttggattgtcactaattcccactgctgtgcaattcacatgcctgtgctttttacctgacactccaagatactacgttatgaagggcgacttggcaagggctactgaggtgttgaagagaagttacactgacacttcggaggaaatcattgaacgtaaggtggaagaacttgttactttgaatcaatctattcctggtaagaatgtccctgaaaaagtctggaataccatcaaagaattgcacacagtaccatctaatctaagggctttgatcattggttgtggtttacaagcaattcaacagtttaccggttggaattcgttgatgtatttctctggtaccatcttcgaaactgtcggtttcaaaaattcttccgctgtttcaatcatcgtgtccggtaccaattttattttcactttagttgcctttttttccattgacaaaataggccgtagaaccatattattgattggattaccaggcatgaccatggctttagtcgtgtgctctattgctttccattttctaggtattaagtttgatggcgctgtcgctgtggtggtttcctccggtttctcctcttggggtattgtgatcatcgtatttattatcgtatttgctgcgttctacgctcttggtatcggtactgttccatggcaacaatcggaactattcccccaaaacgtgagaggtattgggacttcatatgcaactgctacaaactgggctggttcactggttattgcatccacatttttgaccatgttacagaatatcactcctgcaggtacatttgcctttttcgcgggattgtcgtgcttatcaaccattttctgctacttctgttatccagaattatcgggattggagttagaagaggtacaaactattttgaaggacgggttcaacatcaaagcctcgaaagctttggccaagaagagaaaacagcaagttgccagagttcatgaattgaaatatgaaccaactcaagagattatagaggatatataggttaattcaaattaattgatatagttttttaatgagtattgaatctgtttagaaataatggaatattatttttatttatttatttatattattggtcggctcttttcttctgaaggtcaatgacaaaatgatatgaaggaaataatgatttctaaaattttacaacgtaagatatttttacaaaagcctagctcatcttttgtcatgcactattttactcacgcttgaaattaacggccagtccactgcggagtcatttcaaagtcatcctaatcgatctatcgtttttgatagctcattttggagttcgcgattgtcttctgttattcacaactgttttaatttttatttcattctggaactcttcgagttctttgtaaagtctttcatagtagcttactgcatagagctaattaggtttgagttaaggaaaaaaatctatcataagtgtcttgaggtatttactataatgtatacgggaaatattaggtgtgataggctctaggaacgaatattaatattgggggggggaaactggaatgaaattaaacaaaagcaaaaatctaaaagaagaaaaagagagagagagagagagagagagagagagagagatgagggttattgataatataatataataataaaagagaagatagtagaaaaggaagaaagaaaaaaaaaaattaagatgtactttaataaaaagagggaaattctaaaaagtgcgactggaattagaagaatgcaggtattttgttttctctcctatgacggagaaggtaacaaaatcataaaggtaaaataacaaattaattatgatcaaagagaaatgccctttgtaaaccgtggtttgtaaatgcgttggtaactgcagcagatgttaagaaacaaagatggaaaagaaccaaaatcagcttgtaagttc

SEQ ID NO: 30 - DNA, 3279 bp, synthetic construct
  source 1..3279: mol_type = other DNA
atgctttttgataacaaaaatcgcggtgctttaaactcactgaacacaccagatattgcttctttatcaatatcatccatgtcggactatcacgtgtttgattttcccggtaaggacctgcagagagaggaagtgatagatttgctagatcagcaagggtttattcccgacgatttgatcgaacaagaagtagattggttttataactcattgggtattgacgatttgttcttctcgagagaatctccccaattaatctcgaatatcatacattctttgtatgcttcaaagctagatttctttgcgaagtccaaattcaacggaattcagccaaggctattcagcattaaaaacaaaattataactaatgataatcatgccatctttatggaatctaatactggtgtcagcataagcgattctcagcaaaaaaactttaaatttgctagtgacgccgtcggaaacgatactttggagcatggtaaggataccatcaaaaaaaataggattgaaatggatgattcttgtccaccttatgaattagattccgaaattgatgaccttttcctggataacaagtctcaaaaaaactgcagattagtttctttttgggctccagaaagcgaattaaagctaacttttgtttatgagagtgtttaccctaatgatgatccagccggcgtagatatttcctctcaggatttgctgaaaggtgatattgaatcgattagtgataagaccatgtacaaagtttcgtcgaacgaaaataaaaaactatacggtctcttacttaagttggttaaagaaagagaaggtcctgtcattaagactactcgctccgtagaaaataaggatgaaattaggttattagtcgcttacaagcgattcaccactaagcgttattactctgctttgaactctttgttccactattacaagttgaaaccttctaagttctatttagagtcgtttaatgttaaggatgatgacatcattatcttttccgtttatttgaacgagaaccagcaattggaagatgttctacttcacgatgtggaggcagcattgaaacaggttgaaagagaagcttcattgctatacgctatcccaaacaattctttccatgaggtttaccagagacgtcaattctcgcccaaagaagctatatatgctcatattggtgctatattcattaaccattttgttaatcgtttaggctctgattatcaaaaccttttatctcaaatcaccattaagcgtaatgatactactcttttggagattgtagaaaacctaaaaagaaagttaagaaatgaaaccttaactcagcaaactattatcaacatcatgtcgaagcattacactataatttccaagttgtataaaaattttgctcaaattcactattatcataatagtactaaagatatggagaagacattatcttttcaaagactggaaaaagtggagccttttaagaatgaccaagagttcgaagcttacttgaataaattcattccaaatgattcacctgatttgttgatcctgaaaacactgaacatcttcaacaagtctattttgaagacaaatttctttattacaagaaaagtagcaatatcattcagattagatccttccctggtgatgacaaaattcgaatatccagagacaccctatggtatattttttgtcgttggtaatactttcaaagggttccatatcaggttcagagatatcgcaaggggcggtattcgtatagtctgttccaggaatcaggatatttatgatttgaattccaagaacgttattgatgagaactatcaattggcctctactcagcaacgtaaaaataaggatattccagagggtggctctaaaggtgtcatcttattgaacccaggattggtagaacatgaccagacatttgtcgccttttcccaatatgtggatgcaatgattgacattctaatcaacgatccattaaaggaaaactatgtcaaccttttaccaaaggaggaaatattattttttggcccagatgaaggaactgctggtttcgtggattgggcaactaaccatgctcgtgtgaggaactgcccatggtggaaatcatttttgactggaaaatccccatctttgggtggtattccccatgacgaatatggtatgacttctctgggtgttcgtgcttatgttaataaaatttacgaaactttaaacttgacaaattctactgtttacaaattccaaactggtggtccggatggtgatttgggatccaatgaaattcttttatcttcgccaaacgaatgttatttggcaattctggacggttcaggtgtcctgtgtgatcctaaaggtttagataaagatgaattatgccgcttggcacatgaaaggaaaatgatttccgatttcgacacttccaaattatcaaacaacggattttttgtttctgtggatgcaatggatatcatgctaccaaatggtacaattgtagctaacggcacaaccttcagaaacacctttcatactcaaattttcaaatttgtggatcatgtcgacatttttgttccatgcggtggtagaccaaactcaattactctaaataatctacattattttgttgacgaaaagactgggaaatgtaaaattccatatattgtggagggtgccaatctatttataacgcaacctgctaaaaatgctttggaggaacatggctgtattctgttcaaagatgcttctgcaaacaaaggtggtgtcacatcttcatcaatggaagtgttggcctcactagcgcttaacgataacgacttcgtgcacaaatttattggagatgttagtggtgagaggtctgcgttgtacaagtcgtacgttgtagaagtgcagtcaagaattcagaaaaatgctgaattagagtttggtcagttatggaatttgaatcaactaaatggaacccacatttcagaaatttcaaaccaattgtccttcactataaacaaattgaacgacgatctagttgcttctcaagagttgtggctcaatgatctaaaattaagaaactacctattgttggataaaataattccaaaaattctgattgatgttgctgggcctcagtccgtattggaaaacattccagagagctatttgaaagttcttctgtcgagttacttatcaagcacttttgtttaccagaacggtatcgatgttaacattggaaaattcttggaatttattggtgggttaaaaagagaagcggaggcaagtgcttga

SEQ ID NO: 31 - DNA, 3353 bp, synthetic construct
  source 1..3353: mol_type = other DNA
ggcaaacttgaataatgtcgacaatatgaacatcgatagtaagcagaagtccaatgcaatggattcagaattggctaatatcgacaatacaaagaacccattggatattcttgcatcgatggaatctaaaaagaacaccgatgagaactttggtgttgataatgaccaagacatggaccagtttgcaaccaatgacgatttgatggggaacaatcctaactatctaggcagtgacgtggatctgaaggaactgttacagaatagtgaagatgctgatggccgtattgatattcctgaaggtgatatcaacagtttattcaatgaaattgatcttctaatcggcaatgatgaatcatagattggcagttagttttgcaattaatagattaggtaatctgaaatgttcgagtaaaagataagattgatgtcacttgaccataaacagaaacctaacaggaatacgcctctttaccagtctttttttttcttacgtttcgtgatgaatctataggagaagtggcgtgggctaacgaagaagcagagactgaacttaagtaaagaacttaagattagaacgaacagtacgggccctagaaaattcaccactgtcggaaagttgtctacttccgtcggttggaaatacgagtctgttgttgagaagttggaggagaagagaaaggctgaggaagctgagtaccaggagaagaagagagcttacacccagagattagacgcagctagtgccgagtttgcccaaaccgaggagggaaagcagttggccgcctttggttactaaatagtaaagtagggtatcttcaactaatagtatactaaccatctgaaataaccaccgttcctgtatttgttttttctgagactaaagagcctaggaaattcttcctcaggattttgcgttccatccaacatctgtgcgcaaactaaaagttccgagtctgacatctaccatcgctagaccctatgtaataccaatctcgcgtccgaagttttaactttcagtccttaaaacttcagagtattggttgtagtttccggatctgaggggtcgtattgaagacaaaaaaaagacggagctgcctccacagcgcgaaacgtcaaccctaacaccaaccataatttgcaatcaccatggggacaagtttcagcagtcaatgggtaattcagacgatgatacgctatcaatttgctaagctcaatgatgatttagctggcttcaccgaaaggtctttcattgatgtactctgctgttcattcgtattttatctctctcgttggacaatgcccgggtactcccggaacaagggagtcttccagccaagctgtacacagtgaaaaatagaaatacacctttgaaatcaagacgcgcgttggccaatcacaagacttaatcggtgcaaagaaggattaccaaaattttttttcccaaaatcgctatatagaaataatggaggaaaaagggttaatataaaggagaattcccccgtttttctccccttttcttttcttcttcaggctttcttacaaatctataatattccaaaatggctgacaacaacaagtctaacttcttcgtcgacttcatgttgtacattttcgatttgggtaacgttattgttgatattgatttcaacagagttttgggtgcttggtctgatttgactagaattccattagcttctttgaagaagtctttccacatgggtgaagctttccatcaacatgaaagaggtgaaatttctgatgaagctttcgctgaagctttgtgtcatgaaatggctttgccattgtcttacgaacaattctctcatggttggcaagctgttttcgttgctttgagacctgaagttattgctattatgcataagttgagagaacaaggtcatagagttgttgttttgtctaacactaatagattgcatactactttctggccagaagaatacccagaaattagagatgctgctgatcatatctacttgtctcaagatttgggtatgagaaagccagaagctagaatctaccaacatgttttgcaagctgaaggtttctctccatctgatactgttttcttcgatgataacgctgataacattgaaggtgctaaccaattgggtattacttctattttagttaaggataagactactattccagattacttcgctaaggttttgtgttaaacgggaagtctttacagttttagttaggagcccttatatatgacagtaatgctagtacgttttgttttgtttaattaataacttagtttatgttagcctagtatagactccatcaattttttttgttattacgtaagccgcgatgataatatctgatgaaaaattcctatcagaaaataatttatcaaaagtttcatgcgatatgagactaagtagaatagggactcccaaagtgtcagtcacaagggtcattcccgttcgtaatgtggtgatagcgaggagaaaacctgtcagagcaagtaacaccgacgcaaagacatggctaatgaaagaagagcagagaagaataagacagaaggagcaggagatgaaacaaaggctagaggaactagaaaggttcaaaacaaaagtacagaaatcatatataaggaaagaggataggcatttggcacaagagatagaaaaggatcttgacataatcactgatgattacaatttggttagattagttagtatgcatcgcgcgatcagaatttacctaccttactccataagcgcagagaaatatcatccattctatgaagagtgtacttgtaacaggaggagccactgtcacatttgttgcgctactccaattgactctcaatgaaaagtttatttctgccttgaagaaaaacaatttcgataaacttgttgttcagtatggaactcaacccacaggtgaatcactatttctgtcgctgatcaacaaactaaccgatgaagattataagaagtctcaattaggtcagctatacaacataaagctaaaggatggctttttaatccaaggattgagctttgatactgatttcgtcaagaattacacgtccaaagttgatctcgtgatctcacatggaggaactggctctattctagatactctgagagcaggtaaaaagttggtggttgttgtaaacgatacattggccgataatcaccaactagagctcactgaaaaatttgcagaaagagaagttttgggctattgtcggaaaaacacggtagaggagctgattgatcaagtgaatcaagccgaatcaagagagtttaaaagattggcgcctagcaagggaagaatcatacaagatgttatattgaataatattattaagc

SEQ ID NO: 32 - protein, 575 aa, synthetic construct
MIKKLSLCALSVLAALPVGTVAFAADGDMQLQQVLMLSRHNLRAPLADNGSVLEQSTKKSWPQWDVPGGQLTTKGGVLEIYMGNYTRQWLAQQGLVQNGSCPDSNNVFVYANSLQRTVATAQFFVNGAFPGCDVAVTHQDAMGTMDPIFNPVITDGSEAFNKQALADMAAANGKLALKPAFQRLEKIVDYKSSPACNNKKQCDLSSGQNSFSAENGKEPNVSGPLKVGNSLIDAFTLQYYEGFPLDQVAWGQIKTPEQWKELSAIKNGYQDTLFTSPTIAREVAAPLVDYIRSQLVDQDKANAPKVTLMVGHDSNIASLLSALQVKPYELPDTYEKTPIGGQVVFERWHDAKNDKDLLKVEYVYQTADQLRDADVLSLKNPPKRVTLQLTGCQTDANGYCSWDQFSQALNSALQGTPMQPAAAAKPAAAQPDSDAAPAAAAANSATDKPADNAKADKADADKAKAEKAEADKAAAEKAKAEKADADKAKAEKAEADKAAAEKAKADKAAADKAAAEKAKADKAAADKAAAENAKAEKADAEKAAAEKAKADNATASQAPTAAQSNDAKSVATAAQ

SEQ ID NO: 33 - protein, 199 aa, synthetic construct
MLYIFDLGNVIVDIDFNRVLGAWSDLTRIPLASLKKSFHMGEAFHQHERGEISDEAFAEALCHEMALPLSYEQFSHGWQAVFVALRPEVIAIMHKLREQGHRVVVLSNTNRLHTTFWPEEYPEIRDAADHIYLSQDLGMRKPEARIYQHVLQAEGFSPSDTVFFDDNADNIEGANQLGITSILVKDKTTIPDYFAKVLC

SEQ ID NO: 34 - protein, 242 aa, synthetic construct
MKVMECQTYEELSQIAARITADTIKEKPDAVLGLATGGTPEGTYRQLIRLHQTENLSFQNITTVNLDEYAGLSSDDPNSYHFYMNDRFFQHIDSKPSRHFIPNGNADDLEAECRRYEQLVDSLGDTDIQLLGIGRNGHIGFNEPGTSFKSRTHVVTLNEQTRQANARYFPSIDSVPKKALTMGIQTILSSKRILLLISGKSKAEAVRKLLEGNISEDFPASALHLHSDVTVLIDREAASLRP

SEQ ID NO: 35 - protein, 258 aa, synthetic construct
MIKVLLLDVDGTLLSFETHKVSQSSIDALKKVHDSGIKIVIATGRAASDLHEIDAVPYDGVIALNGAECVLRDGSVIRKVAIPAQDFRKSMELAREFDFAVALELNEGVFVNRLTPTVEQIAGIVEHPVPPVVDIEEMFERKECCQLCFYFDEEAEQKVMPLLSGLSATRWHPLFADVNVAGTSKATGLSLFADYYRVKVSEIMACGDGGNDIPMLKAAGIGVAMGNASEKVQSVADFVTDTVDNSGLYKALKHFGVI

SEQ ID NO: 36 - protein, 511 aa, synthetic construct
MDNPSTNESSNISSIHLESASNRKPTPLIKMIAVASIAAGIQFGWALQLSLLTPYIQLLGVPHKWAANIWLCGPISGMIIQPIVGYYSDRNRSRFGRRRPFIFFGAIAVAVAVFLIGFAADIGHSFGDDLKKKTRPKAVVIFVFGFWILDVANNMLQGPCRAFIGDLAADDHRRMRTGNALFSFFMTVGNVLGYAAGSYRKLFMMLPFTKTEACNEFCANLKTCFFIAIFLLILLSTFALLYVEDIPLPSIESQSQTQTQTQSEPEQQVSCFGEILGAFNGLQKPMWMLMLVTAINWIAWFPFFLFDTDWMGHEVYGGNPGDDAYNRGVRAGAMGLMINAVVLALMSLAVEPLGRFVGGAKRLWGIVNIILAVGLAMTIVITKAAQHERHVSNGNTPSAGISAASFAFFALLGIPLAINFSVPFALASIYSSASGAGQGLSLGVLNIAIVVPQMIVSALSGPWDSLFGGGNLPAFVVGIGAAVISGVLAIIILPTPKATDVAKVPIAGGFH

SEQ ID NO: 37 - protein, 244 aa, synthetic construct
MRQLLLISDLDNTWVGDQQALEHLQEYLGDRRGNFYLAYATGRSYHSARELQKQVGLMEPDYWLTAVGSEIYHPEGLDQHWADYLSEHWQRDILQAIADGFEALKPQSPLEQNPWKISYHLDPQACPTVIDQLTEMLKETGIPVQVIFSSGKDVDLLPQRSNKGNATQYLQQHLAMEPSQTLVCGDSGNDIGLFETSARGVIVRNAQPELLHWYDQWGDSRHYRAQSSHAGAILEAIAHFDFLS

SEQ ID NO: 38 - protein, 720 aa, synthetic construct
MSYSSKYILLISVHGLIRGENLELGRDADTGGQTKYVLELARALVKNPQVARVDLLTRLIKDPKVDADYAQPRELIGDRAQIVRIECGPEEYIAKEMLWDYLDNFADHALDYLKEQPELPDVIHSHYADAGYVGTRLSHQLGIPLVHTGHSLGRSKRTRLLLSGIKADEIESRYNMARRINAEEETLGSAARVITSTHQEIAEQYAQYDYYQPDQMLVIPPGTDLEKFYPPKGNEWETPIVQELQRFLRHPRKPIILALSRPDPRKNIHKLIAAYGQSPQLQAQANLVIVAGNRDDITDLDQGPREVLTDLLLTIDRYDLYGKVAYPKQNQAEDVYALFRLTALSQGVFINPALTEPFGLTLIEAAACGVPIVATEDGGPVDIIKNCQNGYLINPLDEVDIADKLLKVLNDKQQWQFLSESGLEGVKRHYSWPSHVESYLEAINALTQQTSVLKRSDLKRRRTLYYNGALVTSLDQNLLGALQGGLPGDRQTLDELLEVLYQHRKNVGFCIATGRRLDSVLKILREYRIPQPDMLITSMGTEIYSSPDLIPDQSWRNHIDYLWNRNAIVRILGELPGLALQPKEELSAYKISYFYDAAIAPNLEEIRQLLHKGEQTVNTIISFGQFLDILPIRASKGYAVRWLSQQWNIPLEHVFTAGGSGADEDMMRGNTLSVVVANRHHEELSNLGEIEPIYFSEKRYAAGILDGLAHYRFFELLDPV

SEQ ID NO: 39 - protein, 499 aa, synthetic construct
MSTKKHTKTHSTYAFESNTNSVAASQMRNALNKLADSSKLDDAARAKFENELDSFFTLFRRYLVEKSSRTTLEWDKIKSPNPDEVVKYEIISQQPENVSNLSKLAVLKLNGGLGTSMGCVGPKSVIEVREGNTFLDLSVRQIEYLNRQYDSDVPLLLMNSFNTDKDTEHLIKKYSANRIRIRSFNQSRFPRVYKDSLLPVPTEYDSPLDAWYPPGHGDLFESLHVSGELDALIAQGREILFVSNGDNLGATVDLKILNHMIETGAEYIMELTDKTRADVKGGTLISYDGQVRLLEVAQVPKEHIDEFKNIRKFTNFNTNNLWINLKAVKRLIESSNLEMEIIPNQKTITRDGHEINVLQLETACGAAIRHFDGAHGVVVPRSRFLPVKTCSDLLLVKSDLFRLEHGSLKLDPSRFGPNPLIKLGSHFKKVSGFNARIPHIPKIVELDHLTITGNVFLGKDVTLRGTVIIVCSDGHKIDIPNGSILENVVVTGNLQILEH

SEQ ID NO: 40 - protein, 431 aa, synthetic construct
MVSLEKNDHLMLARQLPLKSVALILAGGRGTRLKDLTNKRAKPAVHFGGKFRIIDFALSNCINSGIKRMGVITQYQSHTLVQHIQRGWSFFNEEMNEFVDLLPAQQRMKGENWYRGTADAVTQNLDIIRRYKAEYVVILAGDHIYKQDYSRMLIDHVEKGVRCTVVCMPVPIEEASAFGVMAVDENDKTIEFVEKPANPPSMPNDPSKSLASMGIYVFDADYLYELLEEDDRDENSSHDFGKDLIPKITEAGLAYAHPFPLSCVQSDPDAEPYWRDVGTLEAYWKANLDLASVVDKLDMYDRNWPIRTYNESLPPAKFVQDRSGSHGMTLNSLVSDGCVISGSVVVQSVLFSRVRVNSFCNIDSAVLLPEVWVGRSCRLRRCVIDRACVIPEGMVIGENAEEDARRFYRSEEGIVLVTREMLRKLGHKQER

SEQ ID NO: 41 - protein, 533 aa, synthetic construct
MTEDNIAPITSVKVVTDKCTYKDNELLTKYSYENAVVTKTASGRFDVTPTVQDYVFKLDLKKPEKLGIMLIGLGGNNGSTLVASVLANKHNVEFQTKEGVKQPNYFGSMTQCSTLKLGIDAEGNDVYAPFNSLLPMVSPNDFVVSGWDINNADLYEAMQRSQVLEYDLQQRLKAKMSLVKPLPSIYYPDFIAANQDERANNCINLDEKGNVTTRGKWTHLQRIRRDIQNFKEENALDKVIVLWTANTERYVEVSPGVNDTMENLLQSIKNDHEEIAPSTIFAAASILEGVPYINGSPQNTFVPGLVQLAEHEGTFIAGDDLKSGQTKLKSVLAQFLVDAGIKPVSIASYNHLGNNDGYNLSAPKQFRSKEISKSSVIDDIIASNDILYNDKLGKKVDHCIVIKYMKPVGDSKVAMDEYYSELMLGGHNRISIHNVCEDSLLATPLIIDLLVMTEFCTRVSYKKVDPVKEDAGKFENFYPVLTFLSYWLKAPLTRPGFHPVNGLNKQRTALENFLRLLIGLPSQNELRFEERLL

SEQ ID NO: 42 - protein, 584 aa, synthetic construct
MGIHIPYLTSKTSQSNVGDAVGNADSVEFNSEHDSPSKRGKITLESHEIQRAPASDDEDRIQIKPVNDEDDTSVMITFNQSLSPFIITLTFVASISGFMFGYDTGYISSALISIGTDLDHKVLTYGEKEIVTAATSLGALITSIFAGTAADIFGRKRCLMGSNLMFVIGAILQVSAHTFWQMAVGRLIMGFGVGIGSLIAPLFISEIAPKMIRGRLTVINSLWLTGGQLVAYGCGAGLNYVNNGWRILVGLSLIPTAVQFTCLCFLPDTPRYYVMKGDLARATEVLKRSYTDTSEEIIERKVEELVTLNQSIPGKNVPEKVWNTIKELHTVPSNLRALIIGCGLQAIQQFTGWNSLMYFSGTIFETVGFKNSSAVSIIVSGTNFIFTLVAFFSIDKIGRRTILLIGLPGMTMALVVCSIAFHFLGIKFDGAVAVVVSSGFSSWGIVIIVFIIVFAAFYALGIGTVPWQQSELFPQNVRGIGTSYATATNWAGSLVIASTFLTMLQNITPAGTFAFFAGLSCLSTIFCYFCYPELSGLELEEVQTILKDGFNIKASKALAKKRKQQVARVHELKYEPTQEIIEDI

SEQ ID NO: 43 - protein, 1092 aa, synthetic construct
MLFDNKNRGALNSLNTPDIASLSISSMSDYHVFDFPGKDLQREEVIDLLDQQGFIPDDLIEQEVDWFYNSLGIDDLFFSRESPQLISNIIHSLYASKLDFFAKSKFNGIQPRLFSIKNKIITNDNHAIFMESNTGVSISDSQQKNFKFASDAVGNDTLEHGKDTIKKNRIEMDDSCPPYELDSEIDDLFLDNKSQKNCRLVSFWAPESELKLTFVYESVYPNDDPAGVDISSQDLLKGDIESISDKTMYKVSSNENKKLYGLLLKLVKEREGPVIKTTRSVENKDEIRLLVAYKRFTTKRYYSALNSLFHYYKLKPSKFYLESFNVKDDDIIIFSVYLNENQQLEDVLLHDVEAALKQVEREASLLYAIPNNSFHEVYQRRQFSPKEAIYAHIGAIFINHFVNRLGSDYQNLLSQITIKRNDTTLLEIVENLKRKLRNETLTQQTIINIMSKHYTIISKLYKNFAQIHYYHNSTKDMEKTLSFQRLEKVEPFKNDQEFEAYLNKFIPNDSPDLLILKTLNIFNKSILKTNFFITRKVAISFRLDPSLVMTKFEYPETPYGIFFVVGNTFKGFHIRFRDIARGGIRIVCSRNQDIYDLNSKNVIDENYQLASTQQRKNKDIPEGGSKGVILLNPGLVEHDQTFVAFSQYVDAMIDILINDPLKENYVNLLPKEEILFFGPDEGTAGFVDWATNHARVRNCPWWKSFLTGKSPSLGGIPHDEYGMTSLGVRAYVNKIYETLNLTNSTVYKFQTGGPDGDLGSNEILLSSPNECYLAILDGSGVLCDPKGLDKDELCRLAHERKMISDFDTSKLSNNGFFVSVDAMDIMLPNGTIVANGTTFRNTFHTQIFKFVDHVDIFVPCGGRPNSITLNNLHYFVDEKTGKCKIPYIVEGANLFITQPAKNALEEHGCILFKDASANKGGVTSSSMEVLASLALNDNDFVHKFIGDVSGERSALYKSYVVEVQSRIQKNAELEFGQLWNLNQLNGTHISEISNQLSFTINKLNDDLVASQELWLNDLKLRNYLLLDKIIPKILIDVAGPQSVLENIPESYLKVLLSSYLSSTFVYQNGIDVNIGKFLEFIGGLKREAEASA

SEQ ID NO: 44 - protein, 267 aa, synthetic construct
MHPMLNIAVRAARKAGNLIAKNYETPDAVEASQKGSNDFVTNVDKAAEAVIIDTIRKSYPQHTIITEESGELEGTDQDVQWVIDPLDGTTNFIKRLPHFAVSIAVRIKGRTEVAVVYDPMRNELFTATRGQGAQLNGYRLRGSTARDLDGTILATGFPFKAKQYATTYINIVGKLFNECADFRRTGSAALDLAYVAAGRVDGFFEIGLRPWDFAAGELLVREAGGIVSDFTGGHNYMLTGNIVAGNPRVVKAMLANMRDELSDALKR